European Patent Application EP 4 814 009 A1, published September 30, 2026. Title: Fusion protein specifically binding to Extradomain B of Fibronectin (EDB-FN) and transforming growth factor β (TGFβ) and uses thereof. Applicant: MedPacto Inc. The sequence listing filed with the application follows.

SEQUENCE LISTING (117 sequences)

SEQ ID NO: 1 - protein, 26 aa, synthetic construct
SSSPIQGSWTWENGKWTWKGIIRLEQ

SEQ ID NO: 2 - protein, 116 aa, synthetic construct [sequence omitted]

SEQ ID NO: 3 - protein, 108 aa, synthetic construct [sequence omitted]

SEQ ID NO: 4 - protein, 239 aa, synthetic construct
EVQLLESGGGLVQPGGSLRLSCAASGFTFSSFSMSWVRQAPGKGLEWVSSISGSSGTTYYADSVKGRFTISRDNSKNTLYLQMNSLRAEDTAVYYCAKPFPYFDYWGQGTLVTVSSGGGGSGGGGSGGGGSEIVLTQSPGTLSLSPGERATLSCRASQSVSSSFLAWYQQKPGQAPRLLIYYASSRATGIPDRFSGSGSGTDFTLTISRLEPEDFAVYYCQQTGRIPPTFGQGTKVEIK

SEQ ID NO: 5 - protein, 136 aa, synthetic construct
IPPHVQKSVNNDMIVTDNNGAVKFPQLCKFCDVRFSTCDNQKSCMSNCSITSICEKPQEVCVAVWRKNDENITLETVCHDPKLPYHDFILEDAASPKCIMKEKKKPGETFFMCSCSSDECNDNIIFSEEYNTSNPD

SEQ ID NO: 6 - protein, 121 aa, synthetic construct
QVQLVQSGAEVKKPGSSVKVSCKASGGTFSSYAISWVRQAPGQGLEWMGGIIPIFGTANYAQKFQGRVTITADESTSTAYMELSSLRSEDTAVYYCARGLWEVRALPSVYWGQGTLVTVSS

SEQ ID NO: 7 - protein, 108 aa, synthetic construct
SYELTQPPSVSVAPGQTARITCGANDIGSKSVHWYQQKAGQAPVLVVSEDIIRPSGIPERISGSNSGNTATLTISRVEAGDEADYYCQVWDRDSDQYVFGTGTKVTVL

SEQ ID NO: 8 - protein, 244 aa, synthetic construct
QVQLVQSGAEVKKPGSSVKVSCKASGGTFSSYAISWVRQAPGQGLEWMGGIIPIFGTANYAQKFQGRVTITADESTSTAYMELSSLRSEDTAVYYCARGLWEVRALPSVYWGQGTLVTVSSSSSSGSSSSGSSSSGSYELTQPPSVSVAPGQTARITCGANDIGSKSVHWYQQKAGQAPVLVVSEDIIRPSGIPERISGSNSGNTATLTISRVEAGDEADYYCQVWDRDSDQYVFGTGTKVTVL

SEQ ID NO: 9 - protein, 120 aa, synthetic construct [sequence omitted]

SEQ ID NO: 10 - protein, 111 aa, synthetic construct [sequence omitted]

SEQ ID NO: 11 - protein, 246 aa, synthetic construct
QVQLVQSGVEVKKPGASVKVSCKASGYTFTNYYMYWVRQAPGQGLEWMGGINPSNGGTNFNEKFKNRVTLTTDSSTTTAYMELKSLQFDDTAVYYCARRDYRFDMGFDYWGQGTTVTVSSGGGGSGGGGSGGGGSEIVLTQSPATLSLSPGERATLSCRASKGVSTSGYSYLHWYQQKPGQAPRLLIYLASYLESGVPARFSGSGSGTDFTLTISSLEPEDFAVYYCQHSRDLPLTFGGGTKVEIK

SEQ ID NO: 12 - protein, 229 aa, synthetic construct
ESKYGPPCPPCPAPEFLGGPSVFLFPPKPKDTLMISRTPEVTCVVVDVSQEDPEVQFNWYVDGVEVHNAKTKPREEQFNSTYRVVSVLTVLHQDWLNGKEYKCKVSNKGLPSSIEKTISKAKGQPREPQVYTLPPSQEEMTKNQVSLTCLVKGFYPSDIAVEWESNGQPENNYKTTPPVLDSDGSFFLYSRLTVDKSRWQEGNVFSCSVMHEALHNHYTQKSLSLSLGK

SEQ ID NO: 13 - protein, 225 aa, synthetic construct
THTCPPCPAPELLGGPSVFLFPPKPKDTLMISRTPEVTCVVVDVSHEDPEVKFNWYVDGVEVHNAKTKPREEQYNSTYRVVSVLTVLHQDWLNGKEYKCKVSNKALPAPIEKTISKAKGQPREPQVYTLPPSREEMTKNQVSLTCLVKGFYPSDIAVEWESNGQPENNYKTTPPVLDSDGSFFLYSKLTVDKSRWQQGNVFSCSVMHEALHNHYTQKSLSLSPGK

SEQ ID NO: 14 - protein, 326 aa, synthetic construct
ASTKGPSVFPLAPCSRSTSESTAALGCLVKDYFPEPVTVSWNSGALTSGVHTFPAVLQSSGLYSLSSVVTVPSSSLGTKTYTCNVDHKPSNTKVDKRVESKYGPPCPPCPAPEFLGGPSVFLFPPKPKDTLMISRTPEVTCVVVDVSQEDPEVQFNWYVDGVEVHNAKTKPREEQFNSTYRVVSVLTVLHQDWLNGKEYKCKVSNKGLPSSIEKTISKAKGQPREQVYTLPPSQEEMTKNQVSLTCLVKGFYPSDIAVEWESNGQPENNYKTTPPVLDSDGSFFLYSRLTVDKSRWQEGNVFSCSVMHEALHNHYTQKSLSLSLGK

SEQ ID NO: 15 - protein, 106 aa, synthetic construct
RTVAAPSVFIFPPSDEQLKSGTASVVCLLNNFYPREAKVQWKVDNALQSGNSQESVTEQDSKDSTYSLSSTLTLSKADYEKHKVYACEVTHQGLSSPVTKSFNRGE

SEQ ID NO: 16 - protein, 404 aa, synthetic construct
IPPHVQKSVNNDMIVTDNNGAVKFPQLCKFCDVRFSTCDNQKSCMSNCSITSICEKPQEVCVAVWRKNDENITLETVCHDPKLPYHDFILEDAASPKCIMKEKKKPGETFFMCSCSSDECNDNIIFSEEYNTSNPDGGGESKYGPPCPPCPAPEFLGGPSVFLFPPKPKDTLMISRTPEVTCVVVDVSQEDPEVQFNWYVDGVEVHNAKTKPREEQFNSTYRVVSVLTVLHQDWLNGKEYKCKVSNKGLPSSIEKTISKAKGQPREPQVYTLPPSQEEMTKNQVSLTCLVKGFYPSDIAVEWESNGQPENNYKTTPPVLDSDGSFFLYSRLTVDKSRWQEGNVFSCSVMHEALHNHYTQKSLSLSLGKGGGGSGGGGSSSSPIQGSWTWENGKWTWKGIIRLEQ

SEQ ID NO: 17 - protein, 406 aa, synthetic construct
IPPHVQKSVNNDMIVTDNNGAVKFPQLCKFCDVRFSTCDNQKSCMSNCSITSICEKPQEVCVAVWRKNDENITLETVCHDPKLPYHDFILEDAASPKCIMKEKKKPGETFFMCSCSSDECNDNIIFSEEYNTSNPDGGGGSSSSPIQGSWTWENGKWTWKGIIRLEQGGGGSGGGGSESKYGPPCPPCPAPEFLGGPSVFLFPPKPKDTLMISRTPEVTCVVVDVSQEDPEVQFNWYVDGVEVHNAKTKPREEQFNSTYRVVSVLTVLHQDWLNGKEYKCKVSNKGLPSSIEKTISKAKGQPREPQVYTLPPSQEEMTKNQVSLTCLVKGFYPSDIAVEWESNGQPENNYKTTPPVLDSDGSFFLYSRLTVDKSRWQEGNVFSCSVMHEALHNHYTQKSLSLSLGK

SEQ ID NO: 18 - protein, 406 aa, synthetic construct
SSSPIQGSWTWENGKWTWKGIIRLEQGGGGSIPPHVQKSVNNDMIVTDNNGAVKFPQLCKFCDVRFSTCDNQKSCMSNCSITSICEKPQEVCVAVWRKNDENITLETVCHDPKLPYHDFILEDAASPKCIMKEKKKPGETFFMCSCSSDECNDNIIFSEEYNTSNPDGGGGSGGGGSESKYGPPCPPCPAPEFLGGPSVFLFPPKPKDTLMISRTPEVTCVVVDVSQEDPEVQFNWYVDGVEVHNAKTKPREEQFNSTYRVVSVLTVLHQDWLNGKEYKCKVSNKGLPSSIEKTISKAKGQPREPQVYTLPPSQEEMTKNQVSLTCLVKGFYPSDIAVEWESNGQPENNYKTTPPVLDSDGSFFLYSRLTVDKSRWQEGNVFSCSVMHEALHNHYTQKSLSLSLGK

SEQ ID NO: 19 - protein, 393 aa, synthetic construct
SSSPIQGSWTWENGKWTWKGIIRLEQESKYGPPCPPCPAPEFLGGPSVFLFPPKPKDTLMISRTPEVTCVVVDVSQEDPEVQFNWYVDGVEVHNAKTKPREEQFNSTYRVVSVLTVLHQDWLNGKEYKCKVSNKGLPSSIEKTISKAKGQPREPQVYTLPPSQEEMTKNQVSLTCLVKGFYPSDIAVEWESNGQPENNYKTTPPVLDSDGSFFLYSRLTVDKSRWQEGNVFSCSVMHEALHNHYTQKSLSLSLGKGGGIPPHVQKSVNNDMIVTDNNGAVKFPQLCKFCDVRFSTCDNQKSCMSNCSITSICEKPQEVCVAVWRKNDENITLETVCHDPKLPYHDFILEDAASPKCIMKEKKKPGETFFMCSCSSDECNDNIIFSEEYNTSNP

SEQ ID NO: 20 - protein, 399 aa, synthetic construct
ESKYGPPCPPCPAPEFLGGPSVFLFPPKPKDTLMISRTPEVTCVVVDVSQEDPEVQFNWYVDGVEVHNAKTKPREEQFNSTYRVVSVLTVLHQDWLNGKEYKCKVSNKGLPSSIEKTISKAKGQPREPQVYTLPPSQEEMTKNQVSLTCLVKGFYPSDIAVEWESNGQPENNYKTTPPVLDSDGSFFLYSRLTVDKSRWQEGNVFSCSVMHEALHNHYTQKSLSLSLGKGGGSSSPIQGSWTWENGKWTWKGIIRLEQGGGGSIPPHVQKSVNNDMIVTDNNGAVKFPQLCKFCDVRFSTCDNQKSCMSNCSITSICEKPQEVCVAVWRKNDENITLETVCHDPKLPYHDFILEDAASPKCIMKEKKKPGETFFMCSCSSDECNDNIIFSEEYNTSNPD

SEQ ID NO: 21 - protein, 399 aa, synthetic construct
ESKYGPPCPPCPAPEFLGGPSVFLFPPKPKDTLMISRTPEVTCVVVDVSQEDPEVQFNWYVDGVEVHNAKTKPREEQFNSTYRVVSVLTVLHQDWLNGKEYKCKVSNKGLPSSIEKTISKAKGQPREPQVYTLPPSQEEMTKNQVSLTCLVKGFYPSDIAVEWESNGQPENNYKTTPPVLDSDGSFFLYSRLTVDKSRWQEGNVFSCSVMHEALHNHYTQKSLSLSLGKGGGIPPHVQKSVNNDMIVTDNNGAVKFPQLCKFCDVRFSTCDNQKSCMSNCSITSICEKPQEVCVAVWRKNDENITLETVCHDPKLPYHDFILEDAASPKCIMKEKKKPGETFFMCSCSSDECNDNIIFSEEYNTSNPDGGGGSSSSPIQGSWTWENGKWTWKGIIRLEQ

SEQ ID NO: 22 - protein, 437 aa, synthetic construct
SSSPIQGSWTWENGKWTWKGIIRLEQGGGGSIPPHVQKSVNNDMIVTDNNGAVKFPQLCKFCDVRFSTCDNQKSCMSNCSITSICEKPQEVCVAVWRKNDENITLETVCHDPKLPYHDFILEDAASPKCIMKEKKKPGETFFMCSCSSDECNDNIIFSEEYNTSNPDGGGGSSSSPIQGSWTWENGKWTWKGIIRLEQGGGGSGGGGSESKYGPPCPPCPAPEFLGGPSVFLFPPKPKDTLMISRTPEVTCVVVDVSQEDPEVQFNWYVDGVEVHNAKTKPREEQFNSTYRVVSVLTVLHQDWLNGKEYKCKVSNKGLPSSIEKTISKAKGQPREPQVYTLPPSQEEMTKNQVSLTCLVKGFYPSDIAVEWESNGQPENNYKTTPPVLDSDGSFFLYSRLTVDKSRWQEGNVFSCSVMHEALHNHYTQKSLSLSLGK

SEQ ID NO: 23 - protein, 435 aa, synthetic construct
ESKYGPPCPPCPAPEFLGGPSVFLFPPKPKDTLMISRTPEVTCVVVDVSQEDPEVQFNWYVDGVEVHNAKTKPREEQFNSTYRVVSVLTVLHQDWLNGKEYKCKVSNKGLPSSIEKTISKAKGQPREPQVYTLPPSQEEMTKNQVSLTCLVKGFYPSDIAVEWESNGQPENNYKTTPPVLDSDGSFFLYSRLTVDKSRWQEGNVFSCSVMHEALHNHYTQKSLSLSLGKGGGSSSPIQGSWTWENGKWTWKGIIRLEQGGGGSIPPHVQKSVNNDMIVTDNNGAVKFPQLCKFCDVRFSTCDNQKSCMSNCSITSICEKPQEVCVAVWRKNDENITLETVCHDPKLPYHDFILEDAASPKCIMKEKKKPGETFFMCSYSSDECNDNIIFSEEYNTSNPDGGGGSGGGGSSSSPIQGSWTWENGKWTWKGIIRLEQ

SEQ ID NO: 24 - protein, 471 aa, synthetic construct
SSSPIQGSWTWENGKWTWKGIIRLEQGGGGSGGGGSIPPHVQKSVNNDMIVTDNNGAVKFPQLCKFCDVRFSTCDNQKSCMSNCSITSICEKPQEVCVAVWRKNDENITLETVCHDPKLPYHDFILEDAASPKCIMKEKKKPGETFFMCSCSSDECNDNIIFSEEYNTSNPDGGGGSSSSPIQGSWTWENGKWTWKGIIRLEQGGGGSGGGGSESKYGPPCPPCPAPEFLGGPSVFLFPPKPKDTLMISRTPEVTCVVVDVSQEDPEVQFNWYVDGVEVHNAKTKPREEQFNSTYRVVSVLTVLHQDWLNGKEYKCKVSNKGLPSSIEKTISKAKGQPREPQVYTLPPSQEEMTKNQVSLTCLVKGFYPSDIAVEWESNGQPENNYKTTPPVLDSDGSFFLYSRLTVDKSRWQEGNVFSCSVMHEALHNHYTQKSLSLSLGKGGGSSSPIQGSWTWENGKWTWKGIIRLEQ

SEQ ID NO: 25 - protein, 471 aa, synthetic construct
SSSPIQGSWTWENGKWTWKGIIRLEQGGGGSGGGGSESKYGPPCPPCPAPEFLGGPSVFLFPPKPKDTLMISRTPEVTCVVVDVSQEDPEVQFNWYVDGVEVHNAKTKPREEQFNSTYRVVSVLTVLHQDWLNGKEYKCKVSNKGLPSSIEKTISKAKGQPREPQVYTLPPSQEEMTKNQVSLTCLVKGFYPSDIAVEWESNGQPENNYKTTPPVLDSDGSFFLYSRLTVDKSRWQEGNVFSCSVMHEALHNHYTQKSLSLSLGKGGGSSSPIQGSWTWENGKWTWKGIIRLEQGGGGSIPPHVQKSVNNDMIVTDNNGAVKFPQLCKFCDVRFSTCDNQKSCMSNCSITSICEKPQEVCVAVWRKNDENITLETVCHDPKLPYHDFILEDAASPKCIMKEKKKPGETFFMCSYSSDECNDNIIFSEEYNTSNPDGGGGSGGGGSSSSPIQGSWTWENGKWTWKGIIRLEQ

SEQ ID NO: 26 - protein, 401 aa, synthetic construct
IPPHVQKSVNNDMIVTDNNGAVKFPQLCKFCDVRFSTCDNQKSCMSNCSITSICEKPQEVCVAVWRKNDENITLETVCHDPKLPYHDFILEDAASPKCIMKEKKKPGETFFMCSCSSDECNDNIIFSEEYNTSNPDGGGSSSSPIQGSWTWENGKWTWKGIIRLEQGGGGSGGGGSTHTCPPCPAPELLGGPSVFLFPPKPKDTLMISRTPEVTCVVVDVSHEDPEVKFNWYVDGVEVHNAKTKPREEQYNSTYRVVSVLTVLHQDWLNGKEYKCKVSNKALPAPIEKTISKAKGQPREPQVYTLPPSREEMTKNQVSLTCLVKGFYPSDIAVEWESNGQPENNYKTTPPVLDSDGSFFLYSKLTVDKSRWQQGNVFSCSVMHEALHNHYTQKSLSLSPGK

SEQ ID NO: 27 - protein, 397 aa, synthetic construct
THTCPPCPAPELLGGPSVFLFPPKPKDTLMISRTPEVTCVVVDVSHEDPEVKFNWYVDGVEVHNAKTKPREEQYNSTYRVVSVLTVLHQDWLNGKEYKCKVSNKALPAPIEKTISKAKGQPREPQVYTLPPSREEMTKNQVSLTCLVKGFYPSDIAVEWESNGQPENNYKTTPPVLDSDGSFFLYSKLTVDKSRWQQGNVFSCSVMHEALHNHYTQKSLSLSPGKGGGGSSSSPIQGSWTWENGKWTWKGIIRLEQGGGGSIPPHVQKSVNNDMIVTDNNGAVKFPQLCKFCDVRFSTCDNQKSCMSNCSITSICEKPQEVCVAVWRKNDENITLETVCHDPKLPYHDFILEDAASPKCIMKEKKKPGETFFMCSCSSDECNDNIIFSEEYNTSNPD

SEQ ID NO: 28 - protein, 368 aa, synthetic construct
ESKYGPPCPPCPAPEFLGGPSVFLFPPKPKDTLMISRTPEVTCVVVDVSQEDPEVQFNWYVDGVEVHNAKTKPREEQFNSTYRVVSVLTVLHQDWLNGKEYKCKVSNKGLPSSIEKTISKAKGQPREPQVYTLPPSQEEMTKNQVSLTCLVKGFYPSDIAVEWESNGQPENNYKTTPPVLDSDGSFFLYSRLTVDKSRWQEGNVFSCSVMHEALHNHYTQKSLSLSLGKGGGIPPHVQKSVNNDMIVTDNNGAVKFPQLCKFCDVRFSTCDNQKSCMSNCSITSICEKPQEVCVAVWRKNDENITLETVCHDPKLPYHDFILEDAASPKCIMKEKKKPGETFFMCSCSSDECNDNIIFSEEYNTSNPD

SEQ ID NO: 29 - protein, 588 aa, synthetic construct
EVQLLESGGGLVQPGGSLRLSCAASGFTFSSFSMSWVRQAPGKGLEWVSSISGSSGTTYYADSVKGRFTISRDNSKNTLYLQMNSLRAEDTAVYYCAKPFPYFDYWGQGTLVTVSSASTKGPSVFPLAPCSRSTSESTAALGCLVKDYFPEPVTVSWNSGALTSGVHTFPAVLQSSGLYSLSSVVTVPSSSLGTKTYTCNVDHKPSNTKVDKRVESKYGPPCPPCPAPEFLGGPSVFLFPPKPKDTLMISRTPEVTCVVVDVSQEDPEVQFNWYVDGVEVHNAKTKPREEQFNSTYRVVSVLTVLHQDWLNGKEYKCKVSNKGLPSSIEKTISKAKGQPREQVYTLPPSQEEMTKNQVSLTCLVKGFYPSDIAVEWESNGQPENNYKTTPPVLDSDGSFFLYSRLTVDKSRWQEGNVFSCSVMHEALHNHYTQKSLSLSLGKGGGGSGGGGSIPPHVQKSVNNDMIVTDNNGAVKFPQLCKFCDVRFSTCDNQKSCMSNCSITSICEKPQEVCVAVWRKNDENITLETVCHDPKLPYHDFILEDAASPKCIMKEKKKPGETFFMCSYSSDECNDNIIFSEEYNTSNPD

SEQ ID NO: 30 - protein, 361 aa, synthetic construct
EIVLTQSPGTLSLSPGERATLSCRASQSVSSSFLAWYQQKPGQAPRLLIYYASSRATGIPDRFSGSGSGTDFTLTISRLEPEDFAVYYCQQTGRIPPTFGQGTKVEIKRTVAAPSVFIFPPSDEQLKSGTASVVCLLNNFYPREAKVQWKVDNALQSGNSQESVTEQDSKDSTYSLSSTLTLSKADYEKHKVYACEVTHQGLSSPVTKSFNRGECGGGGSGGGGSIPPHVQKSVNNDMIVTDNNGAVKFPQLCKFCDVRFSTCDNQKSCMSNCSITSICEKPQEVCVAVWRKNDENITLETVCHDPKLPYHDFILEDAASPKCIMKEKKKPGETFFMCSCSSDECNDNIIFSEEYNTSNPD

SEQ ID NO: 31 - protein, 594 aa, synthetic construct
IPPHVQKSVNNDMIVTDNNGAVKFPQLCKFCDVRFSTCDNQKSCMSNCSITSICEKPQEVCVAVWRKNDENITLETVCHDPKLPYHDFILEDAASPKCIMKEKKKPGETFFMCSCSSDECNDNIIFSEEYNTSNPDGGGGSGGGGSGGGGSEVQLLESGGGLVQPGGSLRLSCAASGFTFSSFSMSWVRQAPGKGLEWVSSISGSSGTTYYADSVKGRFTISRDNSKNTLYLQMNSLRAEDTAVYYCAKPFPYFDYWGQGTLVTVSSASTKGPSVFPLAPCSRSTSESTAALGCLVKDYFPEPVTVSWNSGALTSGVHTFPAVLQSSGLYSLSSVVTVPSSSLGTKTYTCNVDHKPSNTKVDKRVESKYGPPCPPCPAPEFLGGPSVFLFPPKPKDTLMISRTPEVTCVVVDVSQEDPEVQFNWYVDGVEVHNAKTKPREEQFNSTYRVVSVLTVLHQDWLNGKEYKCKVSNKGLPSSIEKTISKAKGQPREPQVYTLPPSQEEMTKNQVSLTCLVKGFYPSDIAVEWESNGQPENNYKTTPPVLDSDGSFFLYSRLTVDKSRWQEGNVFSCSVMHEALHNHYTQKSLSLSLGK

SEQ ID NO: 32 - protein, 629 aa, synthetic construct
EVQLLESGGGLVQPGGSLRLSCAASGFTFSSFSMSWVRQAPGKGLEWVSSISGSSGTTYYADSVKGRFTISRDNSKNTLYLQMNSLRAEDTAVYYCAKPFPYFDYWGQGTLVTVSSGGGGSGGGGSGGGGSEIVLTQSPGTLSLSPGERATLSCRASQSVSSSFLAWYQQKPGQAPRLLIYYASSRATGIPDRFSGSGSGTDFTLTISRLEPEDFAVYYCQQTGRIPPTFGQGTKVEIKSSSSGSSSSGSSSSGESKYGPPCPPCPAPEFLGGPSVFLFPPKPKDTLMISRTPEVTCVVVDVSQEDPEVQFNWYVDGVEVHNAKTKPREEQFNSTYRVVSVLTVLHQDWLNGKEYKCKVSNKGLPSSIEKTISKAKGQPREPQVYTLPPSQEEMTKNQVSLTCLVKGFYPSDIAVEWESNGQPENNYKTTPPVLDSDGSFFLYSRLTVDKSRWQEGNVFSCSVMHEALHNHYTQKSLSLSLGKGGGGSGGGGSIPPHVQKSVNNDMIVTDNNGAVKFPQLCKFCDVRFSTCDNQKSCMSNCSITSICEKPQEVCVAVWRKNDENITLETVCHDPKLPYHDFILEDAASPKCIMKEKKKPGETFFMCSCSSDECNDNIIFSEEYNTSNPD

SEQ ID NO: 33 - protein, 634 aa, synthetic construct
ESKYGPPCPPCPAPEFLGGPSVFLFPPKPKDTLMISRTPEVTCVVVDVSQEDPEVQFNWYVDGVEVHNAKTKPREEQFNSTYRVVSVLTVLHQDWLNGKEYKCKVSNKGLPSSIEKTISKAKGQPREPQVYTLPPSQEEMTKNQVSLTCLVKGFYPSDIAVEWESNGQPENNYKTTPPVLDSDGSFFLYSRLTVDKSRWQEGNVFSCSVMHEALHNHYTQKSLSLSLGKSSSSGSSSSGSSSSGEVQLLESGGGLVQPGGSLRLSCAASGFTFSSFSMSWVRQAPGKGLEWVSSISGSSGTTYYADSVKGRFTISRDNSKNTLYLQMNSLRAEDTAVYYCAKPFPYFDYWGQGTLVTVSSGGGGSGGGGSGGGGSEIVLTQSPGTLSLSPGERATLSCRASQSVSSSFLAWYQQKPGQAPRLLIYYASSRATGIPDRFSGSGSGTDFTLTISRLEPEDFAVYYCQQTGRIPPTFGQGTKVEIKSSSSGSSSSGSSSSGIPPHVQKSVNNDMIVTDNNGAVKFPQLCKFCDVRFSTCDNQKSCMSNCSITSICEKPQEVCVAVWRKNDENITLETVCHDPKLPYHDFILEDAASPKCIMKEKKKPGETFFMCSCSSDECNDNIIFSEEYNTSNPD

SEQ ID NO: 34 - protein, 634 aa, synthetic construct
EVQLLESGGGLVQPGGSLRLSCAASGFTFSSFSMSWVRQAPGKGLEWVSSISGSSGTTYYADSVKGRFTISRDNSKNTLYLQMNSLRAEDTAVYYCAKPFPYFDYWGQGTLVTVSSGGGGSGGGGSGGGGSEIVLTQSPGTLSLSPGERATLSCRASQSVSSSFLAWYQQKPGQAPRLLIYYASSRATGIPDRFSGSGSGTDFTLTISRLEPEDFAVYYCQQTGRIPPTFGQGTKVEIKSSSSGSSSSGSSSSGIPPHVQKSVNNDMIVTDNNGAVKFPQLCKFCDVRFSTCDNQKSCMSNCSITSICEKPQEVCVAVWRKNDENITLETVCHDPKLPYHDFILEDAASPKCIMKEKKKPGETFFMCSCSSDECNDNIIFSEEYNTSNPDGGGGSGGGGSGGGGSESKYGPPCPPCPAPEFLGGPSVFLFPPKPKDTLMISRTPEVTCVVVDVSQEDPEVQFNWYVDGVEVHNAKTKPREEQFNSTYRVVSVLTVLHQDWLNGKEYKCKVSNKGLPSSIEKTISKAKGQPREPQVYTLPPSQEEMTKNQVSLTCLVKGFYPSDIAVEWESNGQPENNYKTTPPVLDSDGSFFLYSRLTVDKSRWQEGNVFSCSVMHEALHNHYTQKSLSLSLGK

SEQ ID NO: 35 - protein, 634 aa, synthetic construct
ESKYGPPCPPCPAPEFLGGPSVFLFPPKPKDTLMISRTPEVTCVVVDVSQEDPEVQFNWYVDGVEVHNAKTKPREEQFNSTYRVVSVLTVLHQDWLNGKEYKCKVSNKGLPSSIEKTISKAKGQPREPQVYTLPPSQEEMTKNQVSLTCLVKGFYPSDIAVEWESNGQPENNYKTTPPVLDSDGSFFLYSRLTVDKSRWQEGNVFSCSVMHEALHNHYTQKSLSLSLGKSSSSGSSSSGSSSSGIPPHVQKSVNNDMIVTDNNGAVKFPQLCKFCDVRFSTCDNQKSCMSNCSITSICEKPQEVCVAVWRKNDENITLETVCHDPKLPYHDFILEDAASPKCIMKEKKKPGETFFMCSCSSDECNDNIIFSEEYNTSNPDSSSSGSSSSGSSSSGEVQLLESGGGLVQPGGSLRLSCAASGFTFSSFSMSWVRQAPGKGLEWVSSISGSSGTTYYADSVKGRFTISRDNSKNTLYLQMNSLRAEDTAVYYCAKPFPYFDYWGQGTLVTVSSGGGGSGGGGSGGGGSEIVLTQSPGTLSLSPGERATLSCRASQSVSSSFLAWYQQKPGQAPRLLIYYASSRATGIPDRFSGSGSGTDFTLTISRLEPEDFAVYYCQQTGRIPPTFGQGTKVEIK

SEQ ID NO: 36 - protein, 390 aa, synthetic construct
EVQLLESGGGLVQPGGSLRLSCAASGFTFSSFSMSWVRQAPGKGLEWVSSISGSSGTTYYADSVKGRFTISRDNSKNTLYLQMNSLRAEDTAVYYCAKPFPYFDYWGQGTLVTVSSGGGGSGGGGSGGGGSEIVLTQSPGTLSLSPGERATLSCRASQSVSSSFLAWYQQKPGQAPRLLIYYASSRATGIPDRFSGSGSGTDFTLTISRLEPEDFAVYYCQQTGRIPPTFGQGTKVEIKSSSSGSSSSGSSSSGIPPHVQKSVNNDMIVTDNNGAVKFPQLCKFCDVRFSTCDNQKSCMSNCSITSICEKPQEVCVAVWRKNDENITLETVCHDPKLPYHDFILEDAASPKCIMKEKKKPGETFFMCSCSSDECNDNIIFSEEYNTSNPD

SEQ ID NO: 37 - protein, 477 aa, synthetic construct
QVQLVQSGAEVKKPGSSVKVSCKASGGTFSSYAISWVRQAPGQGLEWMGGIIPIFGTANYAQKFQGRVTITADESTSTAYMELSSLRSEDTAVYYCARGLWEVRALPSVYWGQGTLVTVSSASTKGPSVFPLAPCSRSTSESTAALGCLVKDYFPEPVTVSWNSGALTSGVHTFPAVLQSSGLYSLSSVVTVPSSSLGTKTYTCNVDHKPSNTKVDKRVESKYGPPCPPCPAPEFLGGPSVFLFPPKPKDTLMISRTPEVTCVVVDVSQEDPEVQFNWYVDGVEVHNAKTKPREEQFNSTYRVVSVLTVLHQDWLNGKEYKCKVSNKGLPSSIEKTISKAKGQPREPQVYTLPPSQEEMTKNQVSLTCLVKGFYPSDIAVEWESNGQPENNYKTTPPVLDSDGSFFLYSRLTVDKSRWQEGNVFSCSVMHEALHNHYTQKSLSLSLGKGGGSSSPIQGSWTWENGKWTWKGIIRLEQ

SEQ ID NO: 38 - protein, 244 aa, synthetic construct
SYELTQPPSVSVAPGQTARITCGANDIGSKSVHWYQQKAGQAPVLVVSEDIIRPSGIPERISGSNSGNTATLTISRVEAGDEADYYCQVWDRDSDQYVFGTGTKVTVLRTVAAPSVFIFPPSDEQLKSGTASVVCLLNNFYPREAKVQWKVDNALQSGNSQESVTEQDSKDSTYSLSSTLTLSKADYEKHKVYACEVTHQGLSSPVTKSFNRGECGGGSSSPIQGSWTWENGKWTWKGIIRLEQ

SEQ ID NO: 39 - protein, 489 aa, synthetic construct
SSSPIQGSWTWENGKWTWKGIIRLEQGGGGSGGGGSGGGGSQVQLVQSGAEVKKPGSSVKVSCKASGGTFSSYAISWVRQAPGQGLEWMGGIIPIFGTANYAQKFQGRVTITADESTSTAYMELSSLRSEDTAVYYCARGLWEVRALPSVYWGQGTLVTVSSASTKGPSVFPLAPCSRSTSESTAALGCLVKDYFPEPVTVSWNSGALTSGVHTFPAVLQSSGLYSLSSVVTVPSSSLGTKTYTCNVDHKPSNTKVDKRVESKYGPPCPPCPAPEFLGGPSVFLFPPKPKDTLMISRTPEVTCVVVDVSQEDPEVQFNWYVDGVEVHNAKTKPREEQFNSTYRVVSVLTVLHQDWLNGKEYKCKVSNKGLPSSIEKTISKAKGQPREPQVYTLPPSQEEMTKNQVSLTCLVKGFYPSDIAVEWESNGQPENNYKTTPPVLDSDGSFFLYSRLTVDKSRWQEGNVFSCSVMHEALHNHYTQKSLSLSLGK

SEQ ID NO: 40 - protein, 517 aa, synthetic construct
QVQLVQSGAEVKKPGSSVKVSCKASGGTFSSYAISWVRQAPGQGLEWMGGIIPIFGTANYAQKFQGRVTITADESTSTAYMELSSLRSEDTAVYYCARGLWEVRALPSVYWGQGTLVTVSSSSSSGSSSSGSSSSGSYELTQPPSVSVAPGQTARITCGANDIGSKSVHWYQQKAGQAPVLVVSEDIIRPSGIPERISGSNSGNTATLTISRVEAGDEADYYCQVWDRDSDQYVFGTGTKVTVLGGGSSSPIQGSWTWENGKWTWKGIIRLEQGGGGSGGGGSGGGGSESKYGPPCPPCPAPEFLGGPSVFLFPPKPKDTLMISRTPEVTCVVVDVSQEDPEVQFNWYVDGVEVHNAKTKPREEQFNSTYRVVSVLTVLHQDWLNGKEYKCKVSNKGLPSSIEKTISKAKGQPREPQVYTLPPSQEEMTKNQVSLTCLVKGFYPSDIAVEWESNGQPENNYKTTPPVLDSDGSFFLYSRLTVDKSRWQEGNVFSCSVMHEALHNHYTQKSLSLSLGK

SEQ ID NO: 41 - protein, 529 aa, synthetic construct
SSSPIQGSWTWENGKWTWKGIIRLEQGGGGSGGGGSGGGGSQVQLVQSGAEVKKPGSSVKVSCKASGGTFSSYAISWVRQAPGQGLEWMGGIIPIFGTANYAQKFQGRVTITADESTSTAYMELSSLRSEDTAVYYCARGLWEVRALPSVYWGQGTLVTVSSSSSSGSSSSGSSSSGSYELTQPPSVSVAPGQTARITCGANDIGSKSVHWYQQKAGQAPVLVVSEDIIRPSGIPERISGSNSGNTATLTISRVEAGDEADYYCQVWDRDSDQYVFGTGTKVTVLGGGGSGGGGSGGGGSESKYGPPCPPCPAPEFLGGPSVFLFPPKPKDTLMISRTPEVTCVVVDVSQEDPEVQFNWYVDGVEVHNAKTKPREEQFNSTYRVVSVLTVLHQDWLNGKEYKCKVSNKGLPSSIEKTISKAKGQPREPQVYTLPPSQEEMTKNQVSLTCLVKGFYPSDIAVEWESNGQPENNYKTTPPVLDSDGSFFLYSRLTVDKSRWQEGNVFSCSVMHEALHNHYTQKSLSLSLGK

SEQ ID NO: 42 - protein, 517 aa, synthetic construct
ESKYGPPCPPCPAPEFLGGPSVFLFPPKPKDTLMISRTPEVTCVVVDVSQEDPEVQFNWYVDGVEVHNAKTKPREEQFNSTYRVVSVLTVLHQDWLNGKEYKCKVSNKGLPSSIEKTISKAKGQPREPQVYTLPPSQEEMTKNQVSLTCLVKGFYPSDIAVEWESNGQPENNYKTTPPVLDSDGSFFLYSRLTVDKSRWQEGNVFSCSVMHEALHNHYTQKSLSLSLGKGGGSSSPIQGSWTWENGKWTWKGIIRLEQGGGGSGGGGSGGGGSQVQLVQSGAEVKKPGSSVKVSCKASGGTFSSYAISWVRQAPGQGLEWMGGIIPIFGTANYAQKFQGRVTITADESTSTAYMELSSLRSEDTAVYYCARGLWEVRALPSVYWGQGTLVTVSSSSSSGSSSSGSSSSGSYELTQPPSVSVAPGQTARITCGANDIGSKSVHWYQQKAGQAPVLVVSEDIIRPSGIPERISGSNSGNTATLTISRVEAGDEADYYCQVWDRDSDQYVFGTGTKVTVL

SEQ ID NO: 43 - protein, 529 aa, synthetic construct
ESKYGPPCPPCPAPEFLGGPSVFLFPPKPKDTLMISRTPEVTCVVVDVSQEDPEVQFNWYVDGVEVHNAKTKPREEQFNSTYRVVSVLTVLHQDWLNGKEYKCKVSNKGLPSSIEKTISKAKGQPREPQVYTLPPSQEEMTKNQVSLTCLVKGFYPSDIAVEWESNGQPENNYKTTPPVLDSDGSFFLYSRLTVDKSRWQEGNVFSCSVMHEALHNHYTQKSLSLSLGKGGGGSGGGGSGGGGSQVQLVQSGAEVKKPGSSVKVSCKASGGTFSSYAISWVRQAPGQGLEWMGGIIPIFGTANYAQKFQGRVTITADESTSTAYMELSSLRSEDTAVYYCARGLWEVRALPSVYWGQGTLVTVSSSSSSGSSSSGSSSSGSYELTQPPSVSVAPGQTARITCGANDIGSKSVHWYQQKAGQAPVLVVSEDIIRPSGIPERISGSNSGNTATLTISRVEAGDEADYYCQVWDRDSDQYVFGTGTKVTVLSSSSGSSSSGSSSSGSSSPIQGSWTWENGKWTWKGIIRLEQ

SEQ ID NO: 44 - protein, 285 aa, synthetic construct
QVQLVQSGAEVKKPGSSVKVSCKASGGTFSSYAISWVRQAPGQGLEWMGGIIPIFGTANYAQKFQGRVTITADESTSTAYMELSSLRSEDTAVYYCARGLWEVRALPSVYWGQGTLVTVSSSSSSGSSSSGSSSSGSYELTQPPSVSVAPGQTARITCGANDIGSKSVHWYQQKAGQAPVLVVSEDIIRPSGIPERISGSNSGNTATLTISRVEAGDEADYYCQVWDRDSDQYVFGTGTKVTVLGGGGSGGGGSGGGGSSSSPIQGSWTWENGKWTWKGIIRLEQ

SEQ ID NO: 45 - protein, 285 aa, synthetic construct
SSSPIQGSWTWENGKWTWKGIIRLEQGGGGSGGGGSGGGGSQVQLVQSGAEVKKPGSSVKVSCKASGGTFSSYAISWVRQAPGQGLEWMGGIIPIFGTANYAQKFQGRVTITADESTSTAYMELSSLRSEDTAVYYCARGLWEVRALPSVYWGQGTLVTVSSSSSSGSSSSGSSSSGSYELTQPPSVSVAPGQTARITCGANDIGSKSVHWYQQKAGQAPVLVVSEDIIRPSGIPERISGSNSGNTATLTISRVEAGDEADYYCQVWDRDSDQYVFGTGTKVTVL

SEQ ID NO: 46 - protein, 701 aa, synthetic construct
EVQLLESGGGLVQPGGSLRLSCAASGFTFSSFSMSWVRQAPGKGLEWVSSISGSSGTTYYADSVKGRFTISRDNSKNTLYLQMNSLRAEDTAVYYCAKPFPYFDYWGQGTLVTVSSASTKGPSVFPLAPCSRSTSESTAALGCLVKDYFPEPVTVSWNSGALTSGVHTFPAVLQSSGLYSLSSVVTVPSSSLGTKTYTCNVDHKPSNTKVDKRVESKYGPPCPPCPAPEFLGGPSVFLFPPKPKDTLMISRTPEVTCVVVDVSQEDPEVQFNWYVDGVEVHNAKTKPREEQFNSTYRVVSVLTVLHQDWLNGKEYKCKVSNKGLPSSIEKTISKAKGQPREQVYTLPPSQEEMTKNQVSLTCLVKGFYPSDIAVEWESNGQPENNYKTTPPVLDSDGSFFLYSRLTVDKSRWQEGNVFSCSVMHEALHNHYTQKSLSLSLGKGGGGSGGGGSGGGGSQVQLVQSGAEVKKPGSSVKVSCKASGGTFSSYAISWVRQAPGQGLEWMGGIIPIFGTANYAQKFQGRVTITADESTSTAYMELSSLRSEDTAVYYCARGLWEVRALPSVYWGQGTLVTVSSSSSSGSSSSGSSSSGSYELTQPPSVSVAPGQTARITCGANDIGSKSVHWYQQKAGQAPVLVVSEDIIRPSGIPERISGSNSGNTATLTISRVEAGDEADYYCQVWDRDSDQYVFGTGTKVTVL

SEQ ID NO: 47 - protein, 702 aa, synthetic construct
QVQLVQSGAEVKKPGSSVKVSCKASGGTFSSYAISWVRQAPGQGLEWMGGIIPIFGTANYAQKFQGRVTITADESTSTAYMELSSLRSEDTAVYYCARGLWEVRALPSVYWGQGTLVTVSSASTKGPSVFPLAPCSRSTSESTAALGCLVKDYFPEPVTVSWNSGALTSGVHTFPAVLQSSGLYSLSSVVTVPSSSLGTKTYTCNVDHKPSNTKVDKRVESKYGPPCPPCPAPEFLGGPSVFLFPPKPKDTLMISRTPEVTCVVVDVSQEDPEVQFNWYVDGVEVHNAKTKPREEQFNSTYRVVSVLTVLHQDWLNGKEYKCKVSNKGLPSSIEKTISKAKGQPREPQVYTLPPSQEEMTKNQVSLTCLVKGFYPSDIAVEWESNGQPENNYKTTPPVLDSDGSFFLYSRLTVDKSRWQEGNVFSCSVMHEALHNHYTQKSLSLSLGKSSSSGSSSSGSSSSGEVQLLESGGGLVQPGGSLRLSCAASGFTFSSFSMSWVRQAPGKGLEWVSSISGSSGTTYYADSVKGRFTISRDNSKNTLYLQMNSLRAEDTAVYYCAKPFPYFDYWGQGTLVTVSSGGGGSGGGGSGGGGSEIVLTQSPGTLSLSPGERATLSCRASQSVSSSFLAWYQQKPGQAPRLLIYYASSRATGIPDRFSGSGSGTDFTLTISRLEPEDFAVYYCQQTGRIPPTFGQGTKVEIK

SEQ ID NO: 48 - protein, 698 aa, synthetic construct
QVQLVQSGAEVKKPGSSVKVSCKASGGTFSSYAISWVRQAPGQGLEWMGGIIPIFGTANYAQKFQGRVTITADESTSTAYMELSSLRSEDTAVYYCARGLWEVRALPSVYWGQGTLVTVSSSSSSGSSSSGSSSSGSYELTQPPSVSVAPGQTARITCGANDIGSKSVHWYQQKAGQAPVLVVSEDIIRPSGIPERISGSNSGNTATLTISRVEAGDEADYYCQVWDRDSDQYVFGTGTKVTVLGGGGGSGGGGSGGGGSEVQLLESGGGLVQPGGSLRLSCAASGFTFSNSAMTWVRQAPGKRLEWVASISGGGTTYYPDSVKGRFTISRDNSKNTLYLQMNSLRAEDTAVYYCARSHYWGQGTLVTVSSASTKGPSVFPLAPCSRSTSESTAALGCLVKDYFPEPVTVSWNSGALTSGVHTFPAVLQSSGLYSLSSVVTVPSSSLGTKTYTCNVDHKPSNTKVDKRVESKYGPPCPPCPAPEFLGGPSVFLFPPKPKDTLMISRTPEVTCVVVDVSQEDPEVQFNWYVDGVEVHNAKTKPREEQFNSTYRVVSVLTVLHQDWLNGKEYKCKVSNKGLPSSIEKTISKAKGQPREPQVYTLPPSQEEMTKNQVSLTCLVKGFYPSDIAVEWESNGQPENNYKTTPPVLDSDGSFFLYSRLTVDKSRWQEGNVFSCSVMHEALHNHYTQKSLSLSLGK

SEQ ID NO: 49 - protein, 698 aa, synthetic construct; identical to SEQ ID NO: 48

SEQ ID NO: 50 - protein, 702 aa, synthetic construct
EVQLLESGGGLVQPGGSLRLSCAASGFTFSSFSMSWVRQAPGKGLEWVSSISGSSGTTYYADSVKGRFTISRDNSKNTLYLQMNSLRAEDTAVYYCAKPFPYFDYWGQGTLVTVSSGGGGSGGGGSGGGGSEIVLTQSPGTLSLSPGERATLSCRASQSVSSSFLAWYQQKPGQAPRLLIYYASSRATGIPDRFSGSGSGTDFTLTISRLEPEDFAVYYCQQTGRIPPTFGQGTKVEIKSSSSGSSSSGSSSSGQVQLVQSGAEVKKPGSSVKVSCKASGGTFSSYAISWVRQAPGQGLEWMGGIIPIFGTANYAQKFQGRVTITADESTSTAYMELSSLRSEDTAVYYCARGLWEVRALPSVYWGQGTLVTVSSASTKGPSVFPLAPCSRSTSESTAALGCLVKDYFPEPVTVSWNSGALTSGVHTFPAVLQSSGLYSLSSVVTVPSSSLGTKTYTCNVDHKPSNTKVDKRVESKYGPPCPPCPAPEFLGGPSVFLFPPKPKDTLMISRTPEVTCVVVDVSQEDPEVQFNWYVDGVEVHNAKTKPREEQFNSTYRVVSVLTVLHQDWLNGKEYKCKVSNKGLPSSIEKTISKAKGQPREPQVYTLPPSQEEMTKNQVSLTCLVKGFYPSDIAVEWESNGQPENNYKTTPPVLDSDGSFFLYSRLTVDKSRWQEGNVFSCSVMHEALHNHYTQKSLSLSLGK

SEQ ID NO: 51 - protein, 743 aa, synthetic construct
EVQLLESGGGLVQPGGSLRLSCAASGFTFSSFSMSWVRQAPGKGLEWVSSISGSSGTTYYADSVKGRFTISRDNSKNTLYLQMNSLRAEDTAVYYCAKPFPYFDYWGQGTLVTVSSGGGGSGGGGSGGGGSEIVLTQSPGTLSLSPGERATLSCRASQSVSSSFLAWYQQKPGQAPRLLIYYASSRATGIPDRFSGSGSGTDFTLTISRLEPEDFAVYYCQQTGRIPPTFGQGTKVEIKSSSSGSSSSGSSSSGQVQLVQSGAEVKKPGSSVKVSCKASGGTFSSYAISWVRQAPGQGLEWMGGIIPIFGTANYAQKFQGRVTITADESTSTAYMELSSLRSEDTAVYYCARGLWEVRALPSVYWGQGTLVTVSSGGGGSGGGGSGGGGSSYELTQPPSVSVAPGQTARITCGANDIGSKSVHWYQQKAGQAPVLVVSEDIIRPSGIPERISGSNSGNTATLTISRVEAGDEADYYCQVWDRDSDQYVFGTGTKVTVLGGGGGSGGGGSGGGGSESKYGPPCPPCPAPEFLGGPSVFLFPPKPKDTLMISRTPEVTCVVVDVSQEDPEVQFNWYVDGVEVHNAKTKPREEQFNSTYRVVSVLTVLHQDWLNGKEYKCKVSNKGLPSSIEKTISKAKGQPREPQVYTLPPSQEEMTKNQVSLTCLVKGFYPSDIAVEWESNGQPENNYKTTPPVLDSDGSFFLYSRLTVDKSRWQEGNVFSCSVMHEALHNHYTQKSLSLSLGK

SEQ ID NO: 52 - protein, 742 aa, synthetic construct
QVQLVQSGAEVKKPGSSVKVSCKASGGTFSSYAISWVRQAPGQGLEWMGGIIPIFGTANYAQKFQGRVTITADESTSTAYMELSSLRSEDTAVYYCARGLWEVRALPSVYWGQGTLVTVSSSSSSGSSSSGSSSSGSYELTQPPSVSVAPGQTARITCGANDIGSKSVHWYQQKAGQAPVLVVSEDIIRPSGIPERISGSNSGNTATLTISRVEAGDEADYYCQVWDRDSDQYVFGTGTKVTVLGGGGSGGGGSGGGGSEVQLLESGGGLVQPGGSLRLSCAASGFTFSSFSMSWVRQAPGKGLEWVSSISGSSGTTYYADSVKGRFTISRDNSKNTLYLQMNSLRAEDTAVYYCAKPFPYFDYWGQGTLVTVSSGGGGSGGGGSGGGGSEIVLTQSPGTLSLSPGERATLSCRASQSVSSSFLAWYQQKPGQAPRLLIYYASSRATGIPDRFSGSGSGTDFTLTISRLEPEDFAVYYCQQTGRIPPTFGQGTKVEIKGGGGSGGGGSGGGGSESKYGPPCPPCPAPEFLGGPSVFLFPPKPKDTLMISRTPEVTCVVVDVSQEDPEVQFNWYVDGVEVHNAKTKPREEQFNSTYRVVSVLTVLHQDWLNGKEYKCKVSNKGLPSSIEKTISKAKGQPREPQVYTLPPSQEEMTKNQVSLTCLVKGFYPSDIAVEWESNGQPENNYKTTPPVLDSDGSFFLYSRLTVDKSRWQEGNVFSCSVMHEALHNHYTQKSLSLSLGK

SEQ ID NO: 53 - protein, 742 aa, synthetic construct
ESKYGPPCPPCPAPEFLGGPSVFLFPPKPKDTLMISRTPEVTCVVVDVSQEDPEVQFNWYVDGVEVHNAKTKPREEQFNSTYRVVSVLTVLHQDWLNGKEYKCKVSNKGLPSSIEKTISKAKGQPREPQVYTLPPSQEEMTKNQVSLTCLVKGFYPSDIAVEWESNGQPENNYKTTPPVLDSDGSFFLYSRLTVDKSRWQEGNVFSCSVMHEALHNHYTQKSLSLSLGKSSSSGSSSSGSSSSGEVQLLESGGGLVQPGGSLRLSCAASGFTFSSFSMSWVRQAPGKGLEWVSSISGSSGTTYYADSVKGRFTISRDNSKNTLYLQMNSLRAEDTAVYYCAKPFPYFDYWGQGTLVTVSSGGGGSGGGGSGGGGSEIVLTQSPGTLSLSPGERATLSCRASQSVSSSFLAWYQQKPGQAPRLLIYYASSRATGIPDRFSGSGSGTDFTLTISRLEPEDFAVYYCQQTGRIPPTFGQGTKVEIKSSSSGSSSSGSSSSGQVQLVQSGAEVKKPGSSVKVSCKASGGTFSSYAISWVRQAPGQGLEWMGGIIPIFGTANYAQKFQGRVTITADESTSTAYMELSSLRSEDTAVYYCARGLWEVRALPSVYWGQGTLVTVSSSSSSGSSSSGSSSSGSYELTQPPSVSVAPGQTARITCGANDIGSKSVHWYQQKAGQAPVLVVSEDIIRPSGIPERISGSNSGNTATLTISRVEAGDEADYYCQVWDRDSDQYVFGTGTKVTVL

SEQ ID NO: 54 - protein, 742 aa, synthetic construct
ESKYGPPCPPCPAPEFLGGPSVFLFPPKPKDTLMISRTPEVTCVVVDVSQEDPEVQFNWYVDGVEVHNAKTKPREEQFNSTYRVVSVLTVLHQDWLNGKEYKCKVSNKGLPSSIEKTISKAKGQPREPQVYTLPPSQEEMTKNQVSLTCLVKGFYPSDIAVEWESNGQPENNYKTTPPVLDSDGSFFLYSRLTVDKSRWQEGNVFSCSVMHEALHNHYTQKSLSLSLGKGGGGSGGGGSGGGGSQVQLVQSGAEVKKPGSSVKVSCKASGGTFSSYAISWVRQAPGQGLEWMGGIIPIFGTANYAQKFQGRVTITADESTSTAYMELSSLRSEDTAVYYCARGLWEVRALPSVYWGQGTLVTVSSSSSSGSSSSGSSSSGSYELTQPPSVSVAPGQTARITCGANDIGSKSVHWYQQKAGQAPVLVVSEDIIRPSGIPERISGSNSGNTATLTISRVEAGDEADYYCQVWDRDSDQYVFGTGTKVTVLGGGGSGGGGSGGGGSEVQLLESGGGLVQPGGSLRLSCAASGFTFSSFSMSWVRQAPGKGLEWVSSISGSSGTTYYADSVKGRFTISRDNSKNTLYLQMNSLRAEDTAVYYCAKPFPYFDYWGQGTLVTVSSGGGGSGGGGSGGGGSEIVLTQSPGTLSLSPGERATLSCRASQSVSSSFLAWYQQKPGQAPRLLIYYASSRATGIPDRFSGSGSGTDFTLTISRLEPEDFAVYYCQQTGRIPPTFGQGTKVEIK

SEQ ID NO: 55 - protein, 499 aa, synthetic construct
EVQLLESGGGLVQPGGSLRLSCAASGFTFSSFSMSWVRQAPGKGLEWVSSISGSSGTTYYADSVKGRFTISRDNSKNTLYLQMNSLRAEDTAVYYCAKPFPYFDYWGQGTLVTVSSGGGGSGGGGSGGGGSEIVLTQSPGTLSLSPGERATLSCRASQSVSSSFLAWYQQKPGQAPRLLIYYASSRATGIPDRFSGSGSGTDFTLTISRLEPEDFAVYYCQQTGRIPPTFGQGTKVEIKSSSSGSSSSGSSSSGQVQLVQSGAEVKKPGSSVKVSCKASGGTFSSYAISWVRQAPGQGLEWMGGIIPIFGTANYAQKFQGRVTITADESTSTAYMELSSLRSEDTAVYYCARGLWEVRALPSVYWGQGTLVTVSSGGGGSGGGGSGGGGSSYELTQPPSVSVAPGQTARITCGANDIGSKSVHWYQQKAGQAPVLVVSEDIIRPSGIPERISGSNSGNTATLTISRVEAGDEADYYCQVWDRDSDQYVFGTGTKVTVLG

SEQ ID NO: 56 - protein, 498 aa, synthetic construct
QVQLVQSGAEVKKPGSSVKVSCKASGGTFSSYAISWVRQAPGQGLEWMGGIIPIFGTANYAQKFQGRVTITADESTSTAYMELSSLRSEDTAVYYCARGLWEVRALPSVYWGQGTLVTVSSSSSSGSSSSGSSSSGSYELTQPPSVSVAPGQTARITCGANDIGSKSVHWYQQKAGQAPVLVVSEDIIRPSGIPERISGSNSGNTATLTISRVEAGDEADYYCQVWDRDSDQYVFGTGTKVTVLGGGGSGGGGSGGGGSEVQLLESGGGLVQPGGSLRLSCAASGFTFSSFSMSWVRQAPGKGLEWVSSISGSSGTTYYADSVKGRFTISRDNSKNTLYLQMNSLRAEDTAVYYCAKPFPYFDYWGQGTLVTVSSGGGGSGGGGSGGGGSEIVLTQSPGTLSLSPGERATLSCRASQSVSSSFLAWYQQKPGQAPRLLIYYASSRATGIPDRFSGSGSGTDFTLTISRLEPEDFAVYYCQQTGRIPPTFGQGTKVEIK

SEQ ID NO: 57 - protein, 622 aa, synthetic construct
QVQLVQSGVEVKKPGASVKVSCKASGYTFTNYYMYWVRQAPGQGLEWMGGINPSNGGTNFNEKFKNRVTLTTDSSTTTAYMELKSLQFDDTAVYYCARRDYRFDMGFDYWGQGTTVTVSSASTKGPSVFPLAPCSRSTSESTAALGCLVKDYFPEPVTVSWNSGALTSGVHTFPAVLQSSGLYSLSSVVTVPSSSLGTKTYTCNVDHKPSNTKVDKRVESKYGPPCPPCPAPEFLGGPSVFLFPPKPKDTLMISRTPEVTCVVVDVSQEDPEVQFNWYVDGVEVHNAKTKPREEQFNSTYRVVSVLTVLHQDWLNGKEYKCKVSNKGLPSSIEKTISKAKGQPREPQVYTLPPSQEEMTKNQVSLTCLVKGFYPSDIAVEWESNGQPENNYKTTPPVLDSDGSFFLYSRLTVDKSRWQEGNVFSCSVMHEALHNHYTQKSLSLSLGKGGGSSSPIQGSWTWENGKWTWKGIIRLEQGGGGSGGGGSIPPHVQKSVNNDMIVTDNNGAVKFPQLCKFCDVRFSTCDNQKSCMSNCSITSICEKPQEVCVAVWRKNDENITLETVCHDPKLPYHDFILEDAASPKCIMKEKKKPGETFFMCSCSSDECNDNIIFSEEYNTSNPD

SEQ ID NO: 58 - protein, 624 aa, synthetic construct
QVQLVQSGVEVKKPGASVKVSCKASGYTFTNYYMYWVRQAPGQGLEWMGGINPSNGGTNFNEKFKNRVTLTTDSSTTTAYMELKSLQFDDTAVYYCARRDYRFDMGFDYWGQGTTVTVSSASTKGPSVFPLAPCSRSTSESTAALGCLVKDYFPEPVTVSWNSGALTSGVHTFPAVLQSSGLYSLSSVVTVPSSSLGTKTYTCNVDHKPSNTKVDKRVESKYGPPCPPCPAPEFLGGPSVFLFPPKPKDTLMISRTPEVTCVVVDVSQEDPEVQFNWYVDGVEVHNAKTKPREEQFNSTYRVVSVLTVLHQDWLNGKEYKCKVSNKGLPSSIEKTISKAKGQPREPQVYTLPPSQEEMTKNQVSLTCLVKGFYPSDIAVEWESNGQPENNYKTTPPVLDSDGSFFLYSRLTVDKSRWQEGNVFSCSVMHEALHNHYTQKSLSLSLGKGGGGSIPPHVQKSVNNDMIVTDNNGAVKFPQLCKFCDVRFSTCDNQKSCMSNCSITSICEKPQEVCVAVWRKNDENITLETVCHDPKLPYHDFILEDAASPKCIMKEKKKPGETFFMCSYSSDECNDNIIFSEEYNTSNPDGGGGSGGGGSSSSPIQGSWTWENGKWTWKGIIRLEQ

SEQ ID NO: 59 - protein, 393 aa, synthetic construct
EIVLTQSPATLSLSPGERATLSCRASKGVSTSGYSYLHWYQQKPGQAPRLLIYLASYLESGVPARFSGSGSGTDFTLTISSLEPEDFAVYYCQHSRDLPLTFGGGTKVEIKRTVAAPSVFIFPPSDEQLKSGTASVVCLLNNFYPREAKVQWKVDNALQSGNSQESVTEQDSKDSTYSLSSTLTLSKADYEKHKVYACEVTHQGLSSPVTKSFNRGECGGGSSSPIQGSWTWENGKWTWKGIIRLEQGGGGSGGGGSIPPHVQKSVNNDMIVTDNNGAVKFPQLCKFCDVRFSTCDNQKSCMSNCSITSICEKPQEVCVAVWRKNDENITLETVCHDPKLPYHDFILEDAASPKCIMKEKKKPGETFFMCSCSSDECNDNIIFSEEYNTSNPD

SEQ ID NO: 60 - protein, 410 aa, synthetic construct
EIVLTQSPATLSLSPGERATLSCRASKGVSTSGYSYLHWYQQKPGQAPRLLIYLASYLESGVPARFSGSGSGTDFTLTISSLEPEDFAVYYCQHSRDLPLTFGGGTKVEIKRTVAAPSVFIFPPSDEQLKSGTASVVCLLNNFYPREAKVQWKVDNALQSGNSQESVTEQDSKDSTYSLSSTLTLSKADYEKHKVYACEVTHQGLSSPVTKSFNRGECGGGGSGGGGSGGGGSIPPHVQKSVNNDMIVTDNNGAVKFPQLCKFCDVRFSTCDNQKSCMSNCSITSICEKPQEVCVAVWRKNDENITLETVCHDPKLPYHDFILEDAASPKCIMKEKKKPGETFFMCSCSSDECNDNIIFSEEYNTSNPDSSSSGSSSSGSSSSGSSSPIQGSWTWENGKWTWKGIIRLEQ

SEQ ID NO: 61 - protein, 639 aa, synthetic construct
IPPHVQKSVNNDMIVTDNNGAVKFPQLCKFCDVRFSTCDNQKSCMSNCSITSICEKPQEVCVAVWRKNDENITLETVCHDPKLPYHDFILEDAASPKCIMKEKKKPGETFFMCSCSSDECNDNIIFSEEYNTSNPDGGGGSGGGGSGGGGSSSSPIQGSWTWENGKWTWKGIIRLEQSSSSGSSSSGSSSSGQVQLVQSGVEVKKPGASVKVSCKASGYTFTNYYMYWVRQAPGQGLEWMGGINPSNGGTNFNEKFKNRVTLTTDSSTTTAYMELKSLQFDDTAVYYCARRDYRFDMGFDYWGQGTTVTVSSASTKGPSVFPLAPCSRSTSESTAALGCLVKDYFPEPVTVSWNSGALTSGVHTFPAVLQSSGLYSLSSVVTVPSSSLGTKTYTCNVDHKPSNTKVDKRVESKYGPPCPPCPAPEFLGGPSVFLFPPKPKDTLMISRTPEVTCVVVDVSQEDPEVQFNWYVDGVEVHNAKTKPREEQFNSTYRVVSVLTVLHQDWLNGKEYKCKVSNKGLPSSIEKTISKAKGQPREPQVYTLPPSQEEMTKNQVSLTCLVKGFYPSDIAVEWESNGQPENNYKTTPPVLDSDGSFFLYSRLTVDKSRWQEGNVFSCSVMHEALHNHYTQKSLSLSLGK

SEQ ID NO: 62 - protein, 639 aa, synthetic construct
SSSPIQGSWTWENGKWTWKGIIRLEQSSSSGSSSSGSSSSGIPPHVQKSVNNDMIVTDNNGAVKFPQLCKFCDVRFSTCDNQKSCMSNCSITSICEKPQEVCVAVWRKNDENITLETVCHDPKLPYHDFILEDAASPKCIMKEKKKPGETFFMCSCSSDECNDNIIFSEEYNTSNPDGGGGSGGGGSGGGGSQVQLVQSGVEVKKPGASVKVSCKASGYTFTNYYMYWVRQAPGQGLEWMGGINPSNGGTNFNEKFKNRVTLTTDSSTTTAYMELKSLQFDDTAVYYCARRDYRFDMGFDYWGQGTTVTVSSASTKGPSVFPLAPCSRSTSESTAALGCLVKDYFPEPVTVSWNSGALTSGVHTFPAVLQSSGLYSLSSVVTVPSSSLGTKTYTCNVDHKPSNTKVDKRVESKYGPPCPPCPAPEFLGGPSVFLFPPKPKDTLMISRTPEVTCVVVDVSQEDPEVQFNWYVDGVEVHNAKTKPREEQFNSTYRVVSVLTVLHQDWLNGKEYKCKVSNKGLPSSIEKTISKAKGQPREPQVYTLPPSQEEMTKNQVSLTCLVKGFYPSDIAVEWESNGQPENNYKTTPPVLDSDGSFFLYSRLTVDKSRWQEGNVFSCSVMHEALHNHYTQKSLSLSLGK

SEQ ID NO: 63 - protein, 660 aa, synthetic construct
QVQLVQSGVEVKKPGASVKVSCKASGYTFTNYYMYWVRQAPGQGLEWMGGINPSNGGTNFNEKFKNRVTLTTDSSTTTAYMELKSLQFDDTAVYYCARRDYRFDMGFDYWGQGTTVTVSSGGGGSGGGGSGGGGSEIVLTQSPATLSLSPGERATLSCRASKGVSTSGYSYLHWYQQKPGQAPRLLIYLASYLESGVPARFSGSGSGTDFTLTISSLEPEDFAVYYCQHSRDLPLTFGGGTKVEIKSSSSGSSSSGSSSSGESKYGPPCPPCPAPEFLGGPSVFLFPPKPKDTLMISRTPEVTCVVVDVSQEDPEVQFNWYVDGVEVHNAKTKPREEQFNSTYRVVSVLTVLHQDWLNGKEYKCKVSNKGLPSSIEKTISKAKGQPREPQVYTLPPSQEEMTKNQVSLTCLVKGFYPSDIAVEWESNGQPENNYKTTPPVLDSDGSFFLYSRLTVDKSRWQEGNVFSCSVMHEALHNHYTQKSLSLSLGKGGGSSSPIQGSWTWENGKWTWKGIIRLEQGGGGSIPPHVQKSVNNDMIVTDNNGAVKFPQLCKFCDVRFSTCDNQKSCMSNCSITSICEKPQEVCVAVWRKNDENITLETVCHDPKLPYHDFILEDAASPKCIMKEKKKPGETFFMCSCSSDECNDNIIFSEEYNTSNPD

SEQ ID NO: 64 - protein, 667 aa, synthetic construct
QVQLVQSGVEVKKPGASVKVSCKASGYTFTNYYMYWVRQAPGQGLEWMGGINPSNGGTNFNEKFKNRVTLTTDSSTTTAYMELKSLQFDDTAVYYCARRDYRFDMGFDYWGQGTTVTVSSGGGGSGGGGSGGGGSEIVLTQSPATLSLSPGERATLSCRASKGVSTSGYSYLHWYQQKPGQAPRLLIYLASYLESGVPARFSGSGSGTDFTLTISSLEPEDFAVYYCQHSRDLPLTFGGGTKVEIKSSSSGSSSSGSSSSGESKYGPPCPPCPAPEFLGGPSVFLFPPKPKDTLMISRTPEVTCVVVDVSQEDPEVQFNWYVDGVEVHNAKTKPREEQFNSTYRVVSVLTVLHQDWLNGKEYKCKVSNKGLPSSIEKTISKAKGQPREPQVYTLPPSQEEMTKNQVSLTCLVKGFYPSDIAVEWESNGQPENNYKTTPPVLDSDGSFFLYSRLTVDKSRWQEGNVFSCSVMHEALHNHYTQKSLSLSLGKGGGGSIPPHVQKSVNNDMIVTDNNGAVKFPQLCKFCDVRFSTCDNQKSCMSNCSITSICEKPQEVCVAVWRKNDENITLETVCHDPKLPYHDFILEDAASPKCIMKEKKKPGETFFMCSYSSDECNDNIIFSEEYNTSNPDGGGGSGGGGSSSSPIQGSWTWENGKWTWKGIIRLEQ

SEQ ID NO: 65 - protein, 682 aa, synthetic construct
IPPHVQKSVNNDMIVTDNNGAVKFPQLCKFCDVRFSTCDNQKSCMSNCSITSICEKPQEVCVAVWRKNDENITLETVCHDPKLPYHDFILEDAASPKCIMKEKKKPGETFFMCSCSSDECNDNIIFSEEYNTSNPDGGGGSGGGGSGGGGSSSSPIQGSWTWENGKWTWKGIIRLEQSSSSGSSSSGSSSSGESKYGPPCPPCPAPEFLGGPSVFLFPPKPKDTLMISRTPEVTCVVVDVSQEDPEVQFNWYVDGVEVHNAKTKPREEQFNSTYRVVSVLTVLHQDWLNGKEYKCKVSNKGLPSSIEKTISKAKGQPREPQVYTLPPSQEEMTKNQVSLTCLVKGFYPSDIAVEWESNGQPENNYKTTPPVLDSDGSFFLYSRLTVDKSRWQEGNVFSCSVMHEALHNHYTQKSLSLSLGKGGGGSGGGGSGGGGSQVQLVQSGVEVKKPGASVKVSCKASGYTFTNYYMYWVRQAPGQGLEWMGGINPSNGGTNFNEKFKNRVTLTTDSSTTTAYMELKSLQFDDTAVYYCARRDYRFDMGFDYWGQGTTVTVSSGGGGSGGGGSGGGGSEIVLTQSPATLSLSPGERATLSCRASKGVSTSGYSYLHWYQQKPGQAPRLLIYLASYLESGVPARFSGSGSGTDFTLTISSLEPEDFAVYYCQHSRDLPLTFGGGTKVEIK

SEQ ID NO: 66 - protein, 438 aa, synthetic construct
QVQLVQSGVEVKKPGASVKVSCKASGYTFTNYYMYWVRQAPGQGLEWMGGINPSNGGTNFNEKFKNRVTLTTDSSTTTAYMELKSLQFDDTAVYYCARRDYRFDMGFDYWGQGTTVTVSSGGGGSGGGGSGGGGSEIVLTQSPATLSLSPGERATLSCRASKGVSTSGYSYLHWYQQKPGQAPRLLIYLASYLESGVPARFSGSGSGTDFTLTISSLEPEDFAVYYCQHSRDLPLTFGGGTKVEIKSSSSGSSSSGSSSSGSSSPIQGSWTWENGKWTWKGIIRLEQGGGGSGGGGSGGGGSIPPHVQKSVNNDMIVTDNNGAVKFPQLCKFCDVRFSTCDNQKSCMSNCSITSICEKPQEVCVAVWRKNDENITLETVCHDPKLPYHDFILEDAASPKCIMKEKKKPGETFFMCSCSSDECNDNIIFSEEYNTSNPD

SEQ ID NO: 67 - protein, 438 aa, synthetic construct
QVQLVQSGVEVKKPGASVKVSCKASGYTFTNYYMYWVRQAPGQGLEWMGGINPSNGGTNFNEKFKNRVTLTTDSSTTTAYMELKSLQFDDTAVYYCARRDYRFDMGFDYWGQGTTVTVSSGGGGSGGGGSGGGGSEIVLTQSPATLSLSPGERATLSCRASKGVSTSGYSYLHWYQQKPGQAPRLLIYLASYLESGVPARFSGSGSGTDFTLTISSLEPEDFAVYYCQHSRDLPLTFGGGTKVEIKSSSSGSSSSGSSSSGIPPHVQKSVNNDMIVTDNNGAVKFPQLCKFCDVRFSTCDNQKSCMSNCSITSICEKPQEVCVAVWRKNDENITLETVCHDPKLPYHDFILEDAASPKCIMKEKKKPGETFFMCSCSSDECNDNIIFSEEYNTSNPDGGGGSGGGGSGGGGSSSSPIQGSWTWENGKWTWKGIIRLEQ

SEQ ID NO: 68 - protein, 438 aa, synthetic construct
IPPHVQKSVNNDMIVTDNNGAVKFPQLCKFCDVRFSTCDNQKSCMSNCSITSICEKPQEVCVAVWRKNDENITLETVCHDPKLPYHDFILEDAASPKCIMKEKKKPGETFFMCSCSSDECNDNIIFSEEYNTSNPDGGGGSGGGGSGGGGSSSSPIQGSWTWENGKWTWKGIIRLEQSSSSGSSSSGSSSSGQVQLVQSGVEVKKPGASVKVSCKASGYTFTNYYMYWVRQAPGQGLEWMGGINPSNGGTNFNEKFKNRVTLTTDSSTTTAYMELKSLQFDDTAVYYCARRDYRFDMGFDYWGQGTTVTVSSGGGGSGGGGSGGGGSEIVLTQSPATLSLSPGERATLSCRASKGVSTSGYSYLHWYQQKPGQAPRLLIYLASYLESGVPARFSGSGSGTDFTLTISSLEPEDFAVYYCQHSRDLPLTFGGGTKVEIK

SEQ ID NO: 69 - protein, 852 aa, synthetic construct
QVQLVQSGVEVKKPGASVKVSCKASGYTFTNYYMYWVRQAPGQGLEWMGGINPSNGGTNFNEKFKNRVTLTTDSSTTTAYMELKSLQFDDTAVYYCARRDYRFDMGFDYWGQGTTVTVSSASTKGPSVFPLAPCSRSTSESTAALGCLVKDYFPEPVTVSWNSGALTSGVHTFPAVLQSSGLYSLSSVVTVPSSSLGTKTYTCNVDHKPSNTKVDKRVESKYGPPCPPCPAPEFLGGPSVFLFPPKPKDTLMISRTPEVTCVVVDVSQEDPEVQFNWYVDGVEVHNAKTKPREEQFNSTYRVVSVLTVLHQDWLNGKEYKCKVSNKGLPSSIEKTISKAKGQPREPQVYTLPPSQEEMTKNQVSLTCLVKGFYPSDIAVEWESNGQPENNYKTTPPVLDSDGSFFLYSRLTVDKSRWQEGNVFSCSVMHEALHNHYTQKSLSLSLGKSSSSGSSSSGSSSSGEVQLLESGGGLVQPGGSLRLSCAASGFTFSSFSMSWVRQAPGKGLEWVSSISGSSGTTYYADSVKGRFTISRDNSKNTLYLQMNSLRAEDTAVYYCAKPFPYFDYWGQGTLVTVSSGGGGSGGGGSGGGGSEIVLTQSPGTLSLSPGERATLSCRASQSVSSSFLAWYQQKPGQAPRLLIYYASSRATGIPDRFSGSGSGTDFTLTISRLEPEDFAVYYCQQTGRIPPTFGQGTKVEIKSSSSGSSSSGSSSSGIPPHVQKSVNNDMIVTDNNGAVKFPQLCKFCDVRFSTCDNQKSCMSNCSITSICEKPQEVCVAVWRKNDENITLETVCHDPKLPYHDFILEDAASPKCIMKEKKKPGETFFMCSCSSDECNDNIIFSEEYNTSNPD

SEQ ID NO: 70 - protein, 842 aa, synthetic construct
QVQLVQSGVEVKKPGASVKVSCKASGYTFTNYYMYWVRQAPGQGLEWMGGINPSNGGTNFNEKFKNRVTLTTDSSTTTAYMELKSLQFDDTAVYYCARRDYRFDMGFDYWGQGTTVTVSSASTKGPSVFPLAPCSRSTSESTAALGCLVKDYFPEPVTVSWNSGALTSGVHTFPAVLQSSGLYSLSSVVTVPSSSLGTKTYTCNVDHKPSNTKVDKRVESKYGPPCPPCPAPEFLGGPSVFLFPPKPKDTLMISRTPEVTCVVVDVSQEDPEVQFNWYVDGVEVHNAKTKPREEQFNSTYRVVSVLTVLHQDWLNGKEYKCKVSNKGLPSSIEKTISKAKGQPREPQVYTLPPSQEEMTKNQVSLTCLVKGFYPSDIAVEWESNGQPENNYKTTPPVLDSDGSFFLYSRLTVDKSRWQEGNVFSCSVMHEALHNHYTQKSLSLSLGKGGGGSIPPHVQKSVNNDMIVTDNNGAVKFPQLCKFCDVRFSTCDNQKSCMSNCSITSICEKPQEVCVAVWRKNDENITLETVCHDPKLPYHDFILEDAASPKCIMKEKKKPGETFFMCSCSSDECNDNIIFSEEYNTSNPDSSSSGSSSSGSSSSGEVQLLESGGGLVQPGGSLRLSCAASGFTFSSFSMSWVRQAPGKGLEWVSSISGSSGTTYYADSVKGRFTISRDNSKNTLYLQMNSLRAEDTAVYYCAKPFPYFDYWGQGTLVTVSSGGGGSGGGGSGGGGSEIVLTQSPGTLSLSPGERATLSCRASQSVSSSFLAWYQQKPGQAPRLLIYYASSRATGIPDRFSGSGSGTDFTLTISRLEPEDFAVYYCQQTGRIPPTFGQGTKVEIK

SEQ ID NO: 71 - protein, 618 aa, synthetic construct
EIVLTQSPATLSLSPGERATLSCRASKGVSTSGYSYLHWYQQKPGQAPRLLIYLASYLESGVPARFSGSGSGTDFTLTISSLEPEDFAVYYCQHSRDLPLTFGGGTKVEIKRTVAAPSVFIFPPSDEQLKSGTASVVCLLNNFYPREAKVQWKVDNALQSGNSQESVTEQDSKDSTYSLSSTLTLSKADYEKHKVYACEVTHQGLSSPVTKSFNRGECSSSSGSSSSGSSSSGEVQLLESGGGLVQPGGSLRLSCAASGFTFSSFSMSWVRQAPGKGLEWVSSISGSSGTTYYADSVKGRFTISRDNSKNTLYLQMNSLRAEDTAVYYCAKPFPYFDYWGQGTLVTVSSGGGGSGGGGSGGGGSEIVLTQSPGTLSLSPGERATLSCRASQSVSSSFLAWYQQKPGQAPRLLIYYASSRATGIPDRFSGSGSGTDFTLTISRLEPEDFAVYYCQQTGRIPPTFGQGTKVEIKGGGGSGGGGSIPPHVQKSVNNDMIVTDNNGAVKFPQLCKFCDVRFSTCDNQKSCMSNCSITSICEKPQEVCVAVWRKNDENITLETVCHDPKLPYHDFILEDAASPKCIMKEKKKPGETFFMCSCSSDECNDNIIFSEEYNTSNPD

SEQ ID NO: 72 - protein, 618 aa, synthetic construct
EIVLTQSPATLSLSPGERATLSCRASKGVSTSGYSYLHWYQQKPGQAPRLLIYLASYLESGVPARFSGSGSGTDFTLTISSLEPEDFAVYYCQHSRDLPLTFGGGTKVEIKRTVAAPSVFIFPPSDEQLKSGTASVVCLLNNFYPREAKVQWKVDNALQSGNSQESVTEQDSKDSTYSLSSTLTLSKADYEKHKVYACEVTHQGLSSPVTKSFNRGECGGGGSGGGGSIPPHVQKSVNNDMIVTDNNGAVKFPQLCKFCDVRFSTCDNQKSCMSNCSITSICEKPQEVCVAVWRKNDENITLETVCHDPKLPYHDFILEDAASPKCIMKEKKKPGETFFMCSCSSDECNDNIIFSEEYNTSNPDSSSSGSSSSGSSSSGEVQLLESGGGLVQPGGSLRLSCAASGFTFSSFSMSWVRQAPGKGLEWVSSISGSSGTTYYADSVKGRFTISRDNSKNTLYLQMNSLRAEDTAVYYCAKPFPYFDYWGQGTLVTVSSGGGGSGGGGSGGGGSEIVLTQSPGTLSLSPGERATLSCRASQSVSSSFLAWYQQKPGQAPRLLIYYASSRATGIPDRFSGSGSGTDFTLTISRLEPEDFAVYYCQQTGRIPPTFGQGTKVEIK

SEQ ID NO: 73 - protein, 847 aa, synthetic construct
EVQLLESGGGLVQPGGSLRLSCAASGFTFSSFSMSWVRQAPGKGLEWVSSISGSSGTTYYADSVKGRFTISRDNSKNTLYLQMNSLRAEDTAVYYCAKPFPYFDYWGQGTLVTVSSGGGGSGGGGSGGGGSEIVLTQSPGTLSLSPGERATLSCRASQSVSSSFLAWYQQKPGQAPRLLIYYASSRATGIPDRFSGSGSGTDFTLTISRLEPEDFAVYYCQQTGRIPPTFGQGTKVEIKGGGGSGGGGSIPPHVQKSVNNDMIVTDNNGAVKFPQLCKFCDVRFSTCDNQKSCMSNCSITSICEKPQEVCVAVWRKNDENITLETVCHDPKLPYHDFILEDAASPKCIMKEKKKPGETFFMCSCSSDECNDNIIFSEEYNTSNPDSSSSGSSSSGSSSSGQVQLVQSGVEVKKPGASVKVSCKASGYTFTNYYMYWVRQAPGQGLEWMGGINPSNGGTNFNEKFKNRVTLTTDSSTTTAYMELKSLQFDDTAVYYCARRDYRFDMGFDYWGQGTTVTVSSASTKGPSVFPLAPCSRSTSESTAALGCLVKDYFPEPVTVSWNSGALTSGVHTFPAVLQSSGLYSLSSVVTVPSSSLGTKTYTCNVDHKPSNTKVDKRVESKYGPPCPPCPAPEFLGGPSVFLFPPKPKDTLMISRTPEVTCVVVDVSQEDPEVQFNWYVDGVEVHNAKTKPREEQFNSTYRVVSVLTVLHQDWLNGKEYKCKVSNKGLPSSIEKTISKAKGQPREPQVYTLPPSQEEMTKNQVSLTCLVKGFYPSDIAVEWESNGQPENNYKTTPPVLDSDGSFFLYSRLTVDKSRWQEGNVFSCSVMHEALHNHYTQKSLSLSLGK

SEQ ID NO: 74 - protein, 852 aa, synthetic construct
IPPHVQKSVNNDMIVTDNNGAVKFPQLCKFCDVRFSTCDNQKSCMSNCSITSICEKPQEVCVAVWRKNDENITLETVCHDPKLPYHDFILEDAASPKCIMKEKKKPGETFFMCSCSSDECNDNIIFSEEYNTSNPDSSSSGSSSSGSSSSGEVQLLESGGGLVQPGGSLRLSCAASGFTFSSFSMSWVRQAPGKGLEWVSSISGSSGTTYYADSVKGRFTISRDNSKNTLYLQMNSLRAEDTAVYYCAKPFPYFDYWGQGTLVTVSSGGGGSGGGGSGGGGSEIVLTQSPGTLSLSPGERATLSCRASQSVSSSFLAWYQQKPGQAPRLLIYYASSRATGIPDRFSGSGSGTDFTLTISRLEPEDFAVYYCQQTGRIPPTFGQGTKVEIKSSSSGSSSSGSSSSGQVQLVQSGVEVKKPGASVKVSCKASGYTFTNYYMYWVRQAPGQGLEWMGGINPSNGGTNFNEKFKNRVTLTTDSSTTTAYMELKSLQFDDTAVYYCARRDYRFDMGFDYWGQGTTVTVSSASTKGPSVFPLAPCSRSTSESTAALGCLVKDYFPEPVTVSWNSGALTSGVHTFPAVLQSSGLYSLSSVVTVPSSSLGTKTYTCNVDHKPSNTKVDKRVESKYGPPCPPCPAPEFLGGPSVFLFPPKPKDTLMISRTPEVTCVVVDVSQEDPEVQFNWYVDGVEVHNAKTKPREEQFNSTYRVVSVLTVLHQDWLNGKEYKCKVSNKGLPSSIEKTISKAKGQPREPQVYTLPPSQEEMTKNQVSLTCLVKGFYPSDIAVEWESNGQPENNYKTTPPVLDSDGSFFLYSRLTVDKSRWQEGNVFSCSVMHEALHNHYTQKSLSLSLGK

SEQ ID NO: 75 - protein, 890 aa, synthetic construct
QVQLVQSGVEVKKPGASVKVSCKASGYTFTNYYMYWVRQAPGQGLEWMGGINPSNGGTNFNEKFKNRVTLTTDSSTTTAYMELKSLQFDDTAVYYCARRDYRFDMGFDYWGQGTTVTVSSGGGGSGGGGSGGGGSEIVLTQSPATLSLSPGERATLSCRASKGVSTSGYSYLHWYQQKPGQAPRLLIYLASYLESGVPARFSGSGSGTDFTLTISSLEPEDFAVYYCQHSRDLPLTFGGGTKVEIKSSSSGSSSSGSSSSGESKYGPPCPPCPAPEFLGGPSVFLFPPKPKDTLMISRTPEVTCVVVDVSQEDPEVQFNWYVDGVEVHNAKTKPREEQFNSTYRVVSVLTVLHQDWLNGKEYKCKVSNKGLPSSIEKTISKAKGQPREPQVYTLPPSQEEMTKNQVSLTCLVKGFYPSDIAVEWESNGQPENNYKTTPPVLDSDGSFFLYSRLTVDKSRWQEGNVFSCSVMHEALHNHYTQKSLSLSLGKSSSSGSSSSGSSSSGEVQLLESGGGLVQPGGSLRLSCAASGFTFSSFSMSWVRQAPGKGLEWVSSISGSSGTTYYADSVKGRFTISRDNSKNTLYLQMNSLRAEDTAVYYCAKPFPYFDYWGQGTLVTVSSGGGGSGGGGSGGGGSEIVLTQSPGTLSLSPGERATLSCRASQSVSSSFLAWYQQKPGQAPRLLIYYASSRATGIPDRFSGSGSGTDFTLTISRLEPEDFAVYYCQQTGRIPPTFGQGTKVEIKGGGGSGGGGSIPPHVQKSVNNDMIVTDNNGAVKFPQLCKFCDVRFSTCDNQKSCMSNCSITSICEKPQEVCVAVWRKNDENITLETVCHDPKLPYHDFILEDAASPKCIMKEKKKPGETFFMCSCSSDECNDNIIFSEEYNTSNPD

SEQ ID NO: 76 - protein, 890 aa, synthetic construct; identical to SEQ ID NO: 75

SEQ ID NO: 77 - protein, 890 aa, synthetic construct
EVQLLESGGGLVQPGGSLRLSCAASGFTFSSFSMSWVRQAPGKGLEWVSSISGSSGTTYYADSVKGRFTISRDNSKNTLYLQMNSLRAEDTAVYYCAKPFPYFDYWGQGTLVTVSSGGGGSGGGGSGGGGSEIVLTQSPGTLSLSPGERATLSCRASQSVSSSFLAWYQQKPGQAPRLLIYYASSRATGIPDRFSGSGSGTDFTLTISRLEPEDFAVYYCQQTGRIPPTFGQGTKVEIKGGGGSGGGGSIPPHVQKSVNNDMIVTDNNGAVKFPQLCKFCDVRFSTCDNQKSCMSNCSITSICEKPQEVCVAVWRKNDENITLETVCHDPKLPYHDFILEDAASPKCIMKEKKKPGETFFMCSCSSDECNDNIIFSEEYNTSNPDSSSSGSSSSGSSSSGESKYGPPCPPCPAPEFLGGPSVFLFPPKPKDTLMISRTPEVTCVVVDVSQEDPEVQFNWYVDGVEVHNAKTKPREEQFNSTYRVVSVLTVLHQDWLNGKEYKCKVSNKGLPSSIEKTISKAKGQPREPQVYTLPPSQEEMTKNQVSLTCLVKGFYPSDIAVEWESNGQPENNYKTTPPVLDSDGSFFLYSRLTVDKSRWQEGNVFSCSVMHEALHNHYTQKSLSLSLGKSSSSGSSSSGSSSSGQVQLVQSGVEVKKPGASVKVSCKASGYTFTNYYMYWVRQAPGQGLEWMGGINPSNGGTNFNEKFKNRVTLTTDSSTTTAYMELKSLQFDDTAVYYCARRDYRFDMGFDYWGQGTTVTVSSGGGGSGGGGSGGGGSEIVLTQSPATLSLSPGERATLSCRASKGVSTSGYSYLHWYQQKPGQAPRLLIYLASYLESGVPARFSGSGSGTDFTLTISSLEPEDFAVYYCQHSRDLPLTFGGGTKVEIK

SEQ ID NO: 78 - protein, 651 aa, synthetic construct
QVQLVQSGVEVKKPGASVKVSCKASGYTFTNYYMYWVRQAPGQGLEWMGGINPSNGGTNFNEKFKNRVTLTTDSSTTTAYMELKSLQFDDTAVYYCARRDYRFDMGFDYWGQGTTVTVSSGGGGSGGGGSGGGGSEIVLTQSPATLSLSPGERATLSCRASKGVSTSGYSYLHWYQQKPGQAPRLLIYLASYLESGVPARFSGSGSGTDFTLTISSLEPEDFAVYYCQHSRDLPLTFGGGTKVEIKSSSSGSSSSGSSSSGEVQLLESGGGLVQPGGSLRLSCAASGFTFSSFSMSWVRQAPGKGLEWVSSISGSSGTTYYADSVKGRFTISRDNSKNTLYLQMNSLRAEDTAVYYCAKPFPYFDYWGQGTLVTVSSGGGGSGGGGSGGGGSEIVLTQSPGTLSLSPGERATLSCRASQSVSSSFLAWYQQKPGQAPRLLIYYASSRATGIPDRFSGSGSGTDFTLTISRLEPEDFAVYYCQQTGRIPPTFGQGTKVEIKSSSSGSSSSGSSSSGIPPHVQKSVNNDMIVTDNNGAVKFPQLCKFCDVRFSTCDNQKSCMSNCSITSICEKPQEVCVAVWRKNDENITLETVCHDPKLPYHDFILEDAASPKCIMKEKKKPGETFFMCSCSSDECNDNIIFSEEYNTSNPD

SEQ ID NO: 79 - protein, 636 aa, synthetic construct
QVQLVQSGVEVKKPGASVKVSCKASGYTFTNYYMYWVRQAPGQGLEWMGGINPSNGGTNFNEKFKNRVTLTTDSSTTTAYMELKSLQFDDTAVYYCARRDYRFDMGFDYWGQGTTVTVSSGGGGSGGGGSGGGGSEIVLTQSPATLSLSPGERATLSCRASKGVSTSGYSYLHWYQQKPGQAPRLLIYLASYLESGVPARFSGSGSGTDFTLTISSLEPEDFAVYYCQHSRDLPLTFGGGTKVEIKSSSSGSSSSGSSSSGIPPHVQKSVNNDMIVTDNNGAVKFPQLCKFCDVRFSTCDNQKSCMSNCSITSICEKPQEVCVAVWRKNDENITLETVCHDPKLPYHDFILEDAASPKCIMKEKKKPGETFFMCSCSSDECNDNIIFSEEYNTSNPDEVQLLESGGGLVQPGGSLRLSCAASGFTFSSFSMSWVRQAPGKGLEWVSSISGSSGTTYYADSVKGRFTISRDNSKNTLYLQMNSLRAEDTAVYYCAKPFPYFDYWGQGTLVTVSSGGGGSGGGGSGGGGSEIVLTQSPGTLSLSPGERATLSCRASQSVSSSFLAWYQQKPGQAPRLLIYYASSRATGIPDRFSGSGSGTDFTLTISRLEPEDFAVYYCQQTGRIPPTFGQGTKVEIK

SEQ ID NO: 80 - protein, 651 aa, synthetic construct
IPPHVQKSVNNDMIVTDNNGAVKFPQLCKFCDVRFSTCDNQKSCMSNCSITSICEKPQEVCVAVWRKNDENITLETVCHDPKLPYHDFILEDAASPKCIMKEKKKPGETFFMCSCSSDECNDNIIFSEEYNTSNPDSSSSGSSSSGSSSSGQVQLVQSGVEVKKPGASVKVSCKASGYTFTNYYMYWVRQAPGQGLEWMGGINPSNGGTNFNEKFKNRVTLTTDSSTTTAYMELKSLQFDDTAVYYCARRDYRFDMGFDYWGQGTTVTVSSGGGGSGGGGSGGGGSEIVLTQSPATLSLSPGERATLSCRASKGVSTSGYSYLHWYQQKPGQAPRLLIYLASYLESGVPARFSGSGSGTDFTLTISSLEPEDFAVYYCQHSRDLPLTFGGGTKVEIKSSSSGSSSSGSSSSGEVQLLESGGGLVQPGGSLRLSCAASGFTFSSFSMSWVRQAPGKGLEWVSSISGSSGTTYYADSVKGRFTISRDNSKNTLYLQMNSLRAEDTAVYYCAKPFPYFDYWGQGTLVTVSSGGGGSGGGGSGGGGSEIVLTQSPGTLSLSPGERATLSCRASQSVSSSFLAWYQQKPGQAPRLLIYYASSRATGIPDRFSGSGSGTDFTLTISRLEPEDFAVYYCQQTGRIPPTFGQGTKVEIK

SEQ ID NO: 81 - protein, 747 aa, synthetic construct
QVQLVQSGVEVKKPGASVKVSCKASGYTFTNYYMYWVRQAPGQGLEWMGGINPSNGGTNFNEKFKNRVTLTTDSSTTTAYMELKSLQFDDTAVYYCARRDYRFDMGFDYWGQGTTVTVSSASTKGPSVFPLAPCSRSTSESTAALGCLVKDYFPEPVTVSWNSGALTSGVHTFPAVLQSSGLYSLSSVVTVPSSSLGTKTYTCNVDHKPSNTKVDKRVESKYGPPCPPCPAPEFLGGPSVFLFPPKPKDTLMISRTPEVTCVVVDVSQEDPEVQFNWYVDGVEVHNAKTKPREEQFNSTYRVVSVLTVLHQDWLNGKEYKCKVSNKGLPSSIEKTISKAKGQPREPQVYTLPPSQEEMTKNQVSLTCLVKGFYPSDIAVEWESNGQPENNYKTTPPVLDSDGSFFLYSRLTVDKSRWQEGNVFSCSVMHEALHNHYTQKSLSLSLGKSSSSGSSSSGSSSSGSSSPIQGSWTWENGKWTWKGIIRLEQGGGGSGGGGSGGGGSQVQLVQSGAEVKKPGSSVKVSCKASGGTFSSYAISWVRQAPGQGLEWMGGIIPIFGTANYAQKFQGRVTITADESTSTAYMELSSLRSEDTAVYYCARGLWEVRALPSVYWGQGTLVTVSSSSSSGSSSSGSSSSGSYELTQPPSVSVAPGQTARITCGANDIGSKSVHWYQQKAGQAPVLVVSEDIIRPSGIPERISGSNSGNTATLTISRVEAGDEADYYCQVWDRDSDQYVFGTGTKVTVL

SEQ ID NO: 82 - protein, 747 aa, synthetic construct
QVQLVQSGVEVKKPGASVKVSCKASGYTFTNYYMYWVRQAPGQGLEWMGGINPSNGGTNFNEKFKNRVTLTTDSSTTTAYMELKSLQFDDTAVYYCARRDYRFDMGFDYWGQGTTVTVSSASTKGPSVFPLAPCSRSTSESTAALGCLVKDYFPEPVTVSWNSGALTSGVHTFPAVLQSSGLYSLSSVVTVPSSSLGTKTYTCNVDHKPSNTKVDKRVESKYGPPCPPCPAPEFLGGPSVFLFPPKPKDTLMISRTPEVTCVVVDVSQEDPEVQFNWYVDGVEVHNAKTKPREEQFNSTYRVVSVLTVLHQDWLNGKEYKCKVSNKGLPSSIEKTISKAKGQPREPQVYTLPPSQEEMTKNQVSLTCLVKGFYPSDIAVEWESNGQPENNYKTTPPVLDSDGSFFLYSRLTVDKSRWQEGNVFSCSVMHEALHNHYTQKSLSLSLGKGGGGSGGGGSGGGGSQVQLVQSGAEVKKPGSSVKVSCKASGGTFSSYAISWVRQAPGQGLEWMGGIIPIFGTANYAQKFQGRVTITADESTSTAYMELSSLRSEDTAVYYCARGLWEVRALPSVYWGQGTLVTVSSSSSSGSSSSGSSSSGSYELTQPPSVSVAPGQTARITCGANDIGSKSVHWYQQKAGQAPVLVVSEDIIRPSGIPERISGSNSGNTATLTISRVEAGDEADYYCQVWDRDSDQYVFGTGTKVTVLGGGGSGGGGSGGGGSSSSPIQGSWTWENGKWTWKGIIRLEQ

SEQ ID NO: 83 - protein, 518 aa, synthetic construct
EIVLTQSPATLSLSPGERATLSCRASKGVSTSGYSYLHWYQQKPGQAPRLLIYLASYLESGVPARFSGSGSGTDFTLTISSLEPEDFAVYYCQHSRDLPLTFGGGTKVEIKRTVAAPSVFIFPPSDEQLKSGTASVVCLLNNFYPREAKVQWKVDNALQSGNSQESVTEQDSKDSTYSLSSTLTLSKADYEKHKVYACEVTHQGLSSPVTKSFNRGECGGGGSGGGGSGGGGSSSSPIQGSWTWENGKWTWKGIIRLEQGGGGSGGGGSGGGGSQVQLVQSGAEVKKPGSSVKVSCKASGGTFSSYAISWVRQAPGQGLEWMGGIIPIFGTANYAQKFQGRVTITADESTSTAYMELSSLRSEDTAVYYCARGLWEVRALPSVYWGQGTLVTVSSSSSSGSSSSGSSSSGSYELTQPPSVSVAPGQTARITCGANDIGSKSVHWYQQKAGQAPVLVVSEDIIRPSGIPERISGSNSGNTATLTISRVEAGDEADYYCQVWDRDSDQYVFGTGTKVTVL

SEQ ID NO: 84 - protein, 512 aa, synthetic construct
EIVLTQSPATLSLSPGERATLSCRASKGVSTSGYSYLHWYQQKPGQAPRLLIYLASYLESGVPARFSGSGSGTDFTLTISSLEPEDFAVYYCQHSRDLPLTFGGGTKVEIKRTVAAPSVFIFPPSDEQLKSGTASVVCLLNNFYPREAKVQWKVDNALQSGNSQESVTEQDSKDSTYSLSSTLTLSKADYEKHKVYACEVTHQGLSSPVTKSFNRGECGGGGSGGGGSGGGGSQVQLVQSGAEVKKPGSSVKVSCKASGGTFSSYAISWVRQAPGQGLEWMGGIIPIFGTANYAQKFQGRVTITADESTSTAYMELSSLRSEDTAVYYCARGLWEVRALPSVYWGQGTLVTVSSSSSSGSSSSGSSSSGSYELTQPPSVSVAPGQTARITCGANDIGSKSVHWYQQKAGQAPVLVVSEDIIRPSGIPERISGSNSGNTATLTISRVEAGDEADYYCQVWDRDSDQYVFGTGTKVTVLGGGSGGGGSSSSPIQGSWTWENGKWTWKGIIRLEQ

SEQ ID NO: 85 - protein, 741 aa, synthetic construct
QVQLVQSGAEVKKPGSSVKVSCKASGGTFSSYAISWVRQAPGQGLEWMGGIIPIFGTANYAQKFQGRVTITADESTSTAYMELSSLRSEDTAVYYCARGLWEVRALPSVYWGQGTLVTVSSSSSSGSSSSGSSSSGSYELTQPPSVSVAPGQTARITCGANDIGSKSVHWYQQKAGQAPVLVVSEDIIRPSGIPERISGSNSGNTATLTISRVEAGDEADYYCQVWDRDSDQYVFGTGTKVTVLGGGSGGGGSSSSPIQGSWTWENGKWTWKGIIRLEQSSSSGSSSSGSSSSGQVQLVQSGVEVKKPGASVKVSCKASGYTFTNYYMYWVRQAPGQGLEWMGGINPSNGGTNFNEKFKNRVTLTTDSSTTTAYMELKSLQFDDTAVYYCARRDYRFDMGFDYWGQGTTVTVSSASTKGPSVFPLAPCSRSTSESTAALGCLVKDYFPEPVTVSWNSGALTSGVHTFPAVLQSSGLYSLSSVVTVPSSSLGTKTYTCNVDHKPSNTKVDKRVESKYGPPCPPCPAPEFLGGPSVFLFPPKPKDTLMISRTPEVTCVVVDVSQEDPEVQFNWYVDGVEVHNAKTKPREEQFNSTYRVVSVLTVLHQDWLNGKEYKCKVSNKGLPSSIEKTISKAKGQPREPQVYTLPPSQEEMTKNQVSLTCLVKGFYPSDIAVEWESNGQPENNYKTTPPVLDSDGSFFLYSRLTVDKSRWQEGNVFSCSVMHEALHNHYTQKSLSLSLGK

SEQ ID NO: 86 - protein, 747 aa, synthetic construct
SSSPIQGSWTWENGKWTWKGIIRLEQGGGGSGGGGSGGGGSQVQLVQSGAEVKKPGSSVKVSCKASGGTFSSYAISWVRQAPGQGLEWMGGIIPIFGTANYAQKFQGRVTITADESTSTAYMELSSLRSEDTAVYYCARGLWEVRALPSVYWGQGTLVTVSSSSSSGSSSSGSSSSGSYELTQPPSVSVAPGQTARITCGANDIGSKSVHWYQQKAGQAPVLVVSEDIIRPSGIPERISGSNSGNTATLTISRVEAGDEADYYCQVWDRDSDQYVFGTGTKVTVLGGGGSGGGGSGGGGSQVQLVQSGVEVKKPGASVKVSCKASGYTFTNYYMYWVRQAPGQGLEWMGGINPSNGGTNFNEKFKNRVTLTTDSSTTTAYMELKSLQFDDTAVYYCARRDYRFDMGFDYWGQGTTVTVSSASTKGPSVFPLAPCSRSTSESTAALGCLVKDYFPEPVTVSWNSGALTSGVHTFPAVLQSSGLYSLSSVVTVPSSSLGTKTYTCNVDHKPSNTKVDKRVESKYGPPCPPCPAPEFLGGPSVFLFPPKPKDTLMISRTPEVTCVVVDVSQEDPEVQFNWYVDGVEVHNAKTKPREEQFNSTYRVVSVLTVLHQDWLNGKEYKCKVSNKGLPSSIEKTISKAKGQPREPQVYTLPPSQEEMTKNQVSLTCLVKGFYPSDIAVEWESNGQPENNYKTTPPVLDSDGSFFLYSRLTVDKSRWQEGNVFSCSVMHEALHNHYTQKSLSLSLGK

SEQ ID NO: 87 - protein, 785 aa, synthetic construct
QVQLVQSGVEVKKPGASVKVSCKASGYTFTNYYMYWVRQAPGQGLEWMGGINPSNGGTNFNEKFKNRVTLTTDSSTTTAYMELKSLQFDDTAVYYCARRDYRFDMGFDYWGQGTTVTVSSGGGGSGGGGSGGGGSEIVLTQSPATLSLSPGERATLSCRASKGVSTSGYSYLHWYQQKPGQAPRLLIYLASYLESGVPARFSGSGSGTDFTLTISSLEPEDFAVYYCQHSRDLPLTFGGGTKVEIKSSSSGSSSSGSSSSGESKYGPPCPPCPAPEFLGGPSVFLFPPKPKDTLMISRTPEVTCVVVDVSQEDPEVQFNWYVDGVEVHNAKTKPREEQFNSTYRVVSVLTVLHQDWLNGKEYKCKVSNKGLPSSIEKTISKAKGQPREPQVYTLPPSQEEMTKNQVSLTCLVKGFYPSDIAVEWESNGQPENNYKTTPPVLDSDGSFFLYSRLTVDKSRWQEGNVFSCSVMHEALHNHYTQKSLSLSLGKGGGGSGGGGSSSSPIQGSWTWENGKWTWKGIIRLEQGGGGSGGGGSGGGGSQVQLVQSGAEVKKPGSSVKVSCKASGGTFSSYAISWVRQAPGQGLEWMGGIIPIFGTANYAQKFQGRVTITADESTSTAYMELSSLRSEDTAVYYCARGLWEVRALPSVYWGQGTLVTVSSSSSSGSSSSGSSSSGSYELTQPPSVSVAPGQTARITCGANDIGSKSVHWYQQKAGQAPVLVVSEDIIRPSGIPERISGSNSGNTATLTISRVEAGDEADYYCQVWDRDSDQYVFGTGTKVTVL

SEQ ID NO: 88 - protein, 785 aa, synthetic construct
QVQLVQSGVEVKKPGASVKVSCKASGYTFTNYYMYWVRQAPGQGLEWMGGINPSNGGTNFNEKFKNRVTLTTDSSTTTAYMELKSLQFDDTAVYYCARRDYRFDMGFDYWGQGTTVTVSSGGGGSGGGGSGGGGSEIVLTQSPATLSLSPGERATLSCRASKGVSTSGYSYLHWYQQKPGQAPRLLIYLASYLESGVPARFSGSGSGTDFTLTISSLEPEDFAVYYCQHSRDLPLTFGGGTKVEIKSSSSGSSSSGSSSSGESKYGPPCPPCPAPEFLGGPSVFLFPPKPKDTLMISRTPEVTCVVVDVSQEDPEVQFNWYVDGVEVHNAKTKPREEQFNSTYRVVSVLTVLHQDWLNGKEYKCKVSNKGLPSSIEKTISKAKGQPREPQVYTLPPSQEEMTKNQVSLTCLVKGFYPSDIAVEWESNGQPENNYKTTPPVLDSDGSFFLYSRLTVDKSRWQEGNVFSCSVMHEALHNHYTQKSLSLSLGKGGGGSGGGGSGGGGSQVQLVQSGAEVKKPGSSVKVSCKASGGTFSSYAISWVRQAPGQGLEWMGGIIPIFGTANYAQKFQGRVTITADESTSTAYMELSSLRSEDTAVYYCARGLWEVRALPSVYWGQGTLVTVSSSSSSGSSSSGSSSSGSYELTQPPSVSVAPGQTARITCGANDIGSKSVHWYQQKAGQAPVLVVSEDIIRPSGIPERISGSNSGNTATLTISRVEAGDEADYYCQVWDRDSDQYVFGTGTKVTVLGGGGSGGGGSSSSPIQGSWTWENGKWTWKGIIRLEQ

SEQ ID NO: 89 - protein, 785 aa, synthetic construct
QVQLVQSGAEVKKPGSSVKVSCKASGGTFSSYAISWVRQAPGQGLEWMGGIIPIFGTANYAQKFQGRVTITADESTSTAYMELSSLRSEDTAVYYCARGLWEVRALPSVYWGQGTLVTVSSSSSSGSSSSGSSSSGSYELTQPPSVSVAPGQTARITCGANDIGSKSVHWYQQKAGQAPVLVVSEDIIRPSGIPERISGSNSGNTATLTISRVEAGDEADYYCQVWDRDSDQYVFGTGTKVTVLGGGGSGGGGSSSSPIQGSWTWENGKWTWKGIIRLEQGGGGSGGGGSGGGGSESKYGPPCPPCPAPEFLGGPSVFLFPPKPKDTLMISRTPEVTCVVVDVSQEDPEVQFNWYVDGVEVHNAKTKPREEQFNSTYRVVSVLTVLHQDWLNGKEYKCKVSNKGLPSSIEKTISKAKGQPREPQVYTLPPSQEEMTKNQVSLTCLVKGFYPSDIAVEWESNGQPENNYKTTPPVLDSDGSFFLYSRLTVDKSRWQEGNVFSCSVMHEALHNHYTQKSLSLSLGKSSSSGSSSSGSSSSGQVQLVQSGVEVKKPGASVKVSCKASGYTFTNYYMYWVRQAPGQGLEWMGGINPSNGGTNFNEKFKNRVTLTTDSSTTTAYMELKSLQFDDTAVYYCARRDYRFDMGFDYWGQGTTVTVSSGGGGSGGGGSGGGGSEIVLTQSPATLSLSPGERATLSCRASKGVSTSGYSYLHWYQQKPGQAPRLLIYLASYLESGVPARFSGSGSGTDFTLTISSLEPEDFAVYYCQHSRDLPLTFGGGTKVEIK

SEQ ID NO: 90 - protein, 541 aa, synthetic construct
QVQLVQSGVEVKKPGASVKVSCKASGYTFTNYYMYWVRQAPGQGLEWMGGINPSNGGTNFNEKFKNRVTLTTDSSTTTAYMELKSLQFDDTAVYYCARRDYRFDMGFDYWGQGTTVTVSSGGGGSGGGGSGGGGSEIVLTQSPATLSLSPGERATLSCRASKGVSTSGYSYLHWYQQKPGQAPRLLIYLASYLESGVPARFSGSGSGTDFTLTISSLEPEDFAVYYCQHSRDLPLTFGGGTKVEIKGGGGSGGGGSSSSPIQGSWTWENGKWTWKGIIRLEQGGGGSGGGGSGGGGSQVQLVQSGAEVKKPGSSVKVSCKASGGTFSSYAISWVRQAPGQGLEWMGGIIPIFGTANYAQKFQGRVTITADESTSTAYMELSSLRSEDTAVYYCARGLWEVRALPSVYWGQGTLVTVSSSSSSGSSSSGSSSSGSYELTQPPSVSVAPGQTARITCGANDIGSKSVHWYQQKAGQAPVLVVSEDIIRPSGIPERISGSNSGNTATLTISRVEAGDEADYYCQVWDRDSDQYVFGTGTKVTVL

SEQ ID NO: 91 - protein, 541 aa, synthetic construct
QVQLVQSGVEVKKPGASVKVSCKASGYTFTNYYMYWVRQAPGQGLEWMGGINPSNGGTNFNEKFKNRVTLTTDSSTTTAYMELKSLQFDDTAVYYCARRDYRFDMGFDYWGQGTTVTVSSGGGGSGGGGSGGGGSEIVLTQSPATLSLSPGERATLSCRASKGVSTSGYSYLHWYQQKPGQAPRLLIYLASYLESGVPARFSGSGSGTDFTLTISSLEPEDFAVYYCQHSRDLPLTFGGGTKVEIKSSSSGSSSSGSSSSGQVQLVQSGAEVKKPGSSVKVSCKASGGTFSSYAISWVRQAPGQGLEWMGGIIPIFGTANYAQKFQGRVTITADESTSTAYMELSSLRSEDTAVYYCARGLWEVRALPSVYWGQGTLVTVSSSSSSGSSSSGSSSSGSYELTQPPSVSVAPGQTARITCGANDIGSKSVHWYQQKAGQAPVLVVSEDIIRPSGIPERISGSNSGNTATLTISRVEAGDEADYYCQVWDRDSDQYVFGTGTKVTVLGGGGSGGGGSSSSPIQGSWTWENGKWTWKGIIRLEQ

SEQ ID NO: 92 - protein, 541 aa, synthetic construct
QVQLVQSGAEVKKPGSSVKVSCKASGGTFSSYAISWVRQAPGQGLEWMGGIIPIFGTANYAQKFQGRVTITADESTSTAYMELSSLRSEDTAVYYCARGLWEVRALPSVYWGQGTLVTVSSSSSSGSSSSGSSSSGSYELTQPPSVSVAPGQTARITCGANDIGSKSVHWYQQKAGQAPVLVVSEDIIRPSGIPERISGSNSGNTATLTISRVEAGDEADYYCQVWDRDSDQYVFGTGTKVTVLGGGGSGGGGSSSSPIQGSWTWENGKWTWKGIIRLEQSSSSGSSSSGSSSSGQVQLVQSGVEVKKPGASVKVSCKASGYTFTNYYMYWVRQAPGQGLEWMGGINPSNGGTNFNEKFKNRVTLTTDSSTTTAYMELKSLQFDDTAVYYCARRDYRFDMGFDYWGQGTTVTVSSGGGGSGGGGSGGGGSEIVLTQSPATLSLSPGERATLSCRASKGVSTSGYSYLHWYQQKPGQAPRLLIYLASYLESGVPARFSGSGSGTDFTLTISSLEPEDFAVYYCQHSRDLPLTFGGGTKVEIK

SEQ ID NO: 93 - protein, 960 aa, synthetic construct
QVQLVQSGVEVKKPGASVKVSCKASGYTFTNYYMYWVRQAPGQGLEWMGGINPSNGGTNFNEKFKNRVTLTTDSSTTTAYMELKSLQFDDTAVYYCARRDYRFDMGFDYWGQGTTVTVSSASTKGPSVFPLAPCSRSTSESTAALGCLVKDYFPEPVTVSWNSGALTSGVHTFPAVLQSSGLYSLSSVVTVPSSSLGTKTYTCNVDHKPSNTKVDKRVESKYGPPCPPCPAPEFLGGPSVFLFPPKPKDTLMISRTPEVTCVVVDVSQEDPEVQFNWYVDGVEVHNAKTKPREEQFNSTYRVVSVLTVLHQDWLNGKEYKCKVSNKGLPSSIEKTISKAKGQPREPQVYTLPPSQEEMTKNQVSLTCLVKGFYPSDIAVEWESNGQPENNYKTTPPVLDSDGSFFLYSRLTVDKSRWQEGNVFSCSVMHEALHNHYTQKSLSLSLGKSSSSGSSSSGSSSSGEVQLLESGGGLVQPGGSLRLSCAASGFTFSSFSMSWVRQAPGKGLEWVSSISGSSGTTYYADSVKGRFTISRDNSKNTLYLQMNSLRAEDTAVYYCAKPFPYFDYWGQGTLVTVSSGGGGSGGGGSGGGGSEIVLTQSPGTLSLSPGERATLSCRASQSVSSSFLAWYQQKPGQAPRLLIYYASSRATGIPDRFSGSGSGTDFTLTISRLEPEDFAVYYCQQTGRIPPTFGQGTKVEIKSSSSGSSSSGSSSSGQVQLVQSGAEVKKPGSSVKVSCKASGGTFSSYAISWVRQAPGQGLEWMGGIIPIFGTANYAQKFQGRVTITADESTSTAYMELSSLRSEDTAVYYCARGLWEVRALPSVYWGQGTLVTVSSSSSSGSSSSGSSSSGSYELTQPPSVSVAPGQTARITCGANDIGSKSVHWYQQKAGQAPVLVVSEDIIRPSGIPERISGSNSGNTATLTISRVEAGDEADYYCQVWDRDSDQYVFGTGTKVTVL

SEQ ID NO: 94 - protein, 960 aa, synthetic construct
QVQLVQSGVEVKKPGASVKVSCKASGYTFTNYYMYWVRQAPGQGLEWMGGINPSNGGTNFNEKFKNRVTLTTDSSTTTAYMELKSLQFDDTAVYYCARRDYRFDMGFDYWGQGTTVTVSSASTKGPSVFPLAPCSRSTSESTAALGCLVKDYFPEPVTVSWNSGALTSGVHTFPAVLQSSGLYSLSSVVTVPSSSLGTKTYTCNVDHKPSNTKVDKRVESKYGPPCPPCPAPEFLGGPSVFLFPPKPKDTLMISRTPEVTCVVVDVSQEDPEVQFNWYVDGVEVHNAKTKPREEQFNSTYRVVSVLTVLHQDWLNGKEYKCKVSNKGLPSSIEKTISKAKGQPREPQVYTLPPSQEEMTKNQVSLTCLVKGFYPSDIAVEWESNGQPENNYKTTPPVLDSDGSFFLYSRLTVDKSRWQEGNVFSCSVMHEALHNHYTQKSLSLSLGKGGGGSGGGGSGGGGSQVQLVQSGAEVKKPGSSVKVSCKASGGTFSSYAISWVRQAPGQGLEWMGGIIPIFGTANYAQKFQGRVTITADESTSTAYMELSSLRSEDTAVYYCARGLWEVRALPSVYWGQGTLVTVSSSSSSGSSSSGSSSSGSYELTQPPSVSVAPGQTARITCGANDIGSKSVHWYQQKAGQAPVLVVSEDIIRPSGIPERISGSNSGNTATLTISRVEAGDEADYYCQVWDRDSDQYVFGTGTKVTVLSSSSGSSSSGSSSSGEVQLLESGGGLVQPGGSLRLSCAASGFTFSSFSMSWVRQAPGKGLEWVSSISGSSGTTYYADSVKGRFTISRDNSKNTLYLQMNSLRAEDTAVYYCAKPFPYFDYWGQGTLVTVSSGGGGSGGGGSGGGGSEIVLTQSPGTLSLSPGERATLSCRASQSVSSSFLAWYQQKPGQAPRLLIYYASSRATGIPDRFSGSGSGTDFTLTISRLEPEDFAVYYCQQTGRIPPTFGQGTKVEIK

SEQ ID NO: 95 - protein, 731 aa, synthetic construct
EIVLTQSPATLSLSPGERATLSCRASKGVSTSGYSYLHWYQQKPGQAPRLLIYLASYLESGVPARFSGSGSGTDFTLTISSLEPEDFAVYYCQHSRDLPLTFGGGTKVEIKRTVAAPSVFIFPPSDEQLKSGTASVVCLLNNFYPREAKVQWKVDNALQSGNSQESVTEQDSKDSTYSLSSTLTLSKADYEKHKVYACEVTHQGLSSPVTKSFNRGECSSSSGSSSSGSSSSGEVQLLESGGGLVQPGGSLRLSCAASGFTFSSFSMSWVRQAPGKGLEWVSSISGSSGTTYYADSVKGRFTISRDNSKNTLYLQMNSLRAEDTAVYYCAKPFPYFDYWGQGTLVTVSSGGGGSGGGGSGGGGSEIVLTQSPGTLSLSPGERATLSCRASQSVSSSFLAWYQQKPGQAPRLLIYYASSRATGIPDRFSGSGSGTDFTLTISRLEPEDFAVYYCQQTGRIPPTFGQGTKVEIKSSSSGSSSSGSSSSGQVQLVQSGAEVKKPGSSVKVSCKASGGTFSSYAISWVRQAPGQGLEWMGGIIPIFGTANYAQKFQGRVTITADESTSTAYMELSSLRSEDTAVYYCARGLWEVRALPSVYWGQGTLVTVSSSSSSGSSSSGSSSSGSYELTQPPSVSVAPGQTARITCGANDIGSKSVHWYQQKAGQAPVLVVSEDIIRPSGIPERISGSNSGNTATLTISRVEAGDEADYYCQVWDRDSDQYVFGTGTKVTVL

SEQ ID NO: 96 - protein, 731 aa, synthetic construct
EIVLTQSPATLSLSPGERATLSCRASKGVSTSGYSYLHWYQQKPGQAPRLLIYLASYLESGVPARFSGSGSGTDFTLTISSLEPEDFAVYYCQHSRDLPLTFGGGTKVEIKRTVAAPSVFIFPPSDEQLKSGTASVVCLLNNFYPREAKVQWKVDNALQSGNSQESVTEQDSKDSTYSLSSTLTLSKADYEKHKVYACEVTHQGLSSPVTKSFNRGECGGGGSGGGGSGGGGSQVQLVQSGAEVKKPGSSVKVSCKASGGTFSSYAISWVRQAPGQGLEWMGGIIPIFGTANYAQKFQGRVTITADESTSTAYMELSSLRSEDTAVYYCARGLWEVRALPSVYWGQGTLVTVSSSSSSGSSSSGSSSSGSYELTQPPSVSVAPGQTARITCGANDIGSKSVHWYQQKAGQAPVLVVSEDIIRPSGIPERISGSNSGNTATLTISRVEAGDEADYYCQVWDRDSDQYVFGTGTKVTVLSSSSGSSSSGSSSSGEVQLLESGGGLVQPGGSLRLSCAASGFTFSSFSMSWVRQAPGKGLEWVSSISGSSGTTYYADSVKGRFTISRDNSKNTLYLQMNSLRAEDTAVYYCAKPFPYFDYWGQGTLVTVSSGGGGSGGGGSGGGGSEIVLTQSPGTLSLSPGERATLSCRASQSVSSSFLAWYQQKPGQAPRLLIYYASSRATGIPDRFSGSGSGTDFTLTISRLEPEDFAVYYCQQTGRIPPTFGQGTKVEIK

SEQ ID NO: 97 - protein, 960 aa, synthetic construct
EVQLLESGGGLVQPGGSLRLSCAASGFTFSSFSMSWVRQAPGKGLEWVSSISGSSGTTYYADSVKGRFTISRDNSKNTLYLQMNSLRAEDTAVYYCAKPFPYFDYWGQGTLVTVSSGGGGSGGGGSGGGGSEIVLTQSPGTLSLSPGERATLSCRASQSVSSSFLAWYQQKPGQAPRLLIYYASSRATGIPDRFSGSGSGTDFTLTISRLEPEDFAVYYCQQTGRIPPTFGQGTKVEIKSSSSGSSSSGSSSSGQVQLVQSGAEVKKPGSSVKVSCKASGGTFSSYAISWVRQAPGQGLEWMGGIIPIFGTANYAQKFQGRVTITADESTSTAYMELSSLRSEDTAVYYCARGLWEVRALPSVYWGQGTLVTVSSSSSSGSSSSGSSSSGSYELTQPPSVSVAPGQTARITCGANDIGSKSVHWYQQKAGQAPVLVVSEDIIRPSGIPERISGSNSGNTATLTISRVEAGDEADYYCQVWDRDSDQYVFGTGTKVTVLGGGGSGGGGSGGGGSQVQLVQSGVEVKKPGASVKVSCKASGYTFTNYYMYWVRQAPGQGLEWMGGINPSNGGTNFNEKFKNRVTLTTDSSTTTAYMELKSLQFDDTAVYYCARRDYRFDMGFDYWGQGTTVTVSSASTKGPSVFPLAPCSRSTSESTAALGCLVKDYFPEPVTVSWNSGALTSGVHTFPAVLQSSGLYSLSSVVTVPSSSLGTKTYTCNVDHKPSNTKVDKRVESKYGPPCPPCPAPEFLGGPSVFLFPPKPKDTLMISRTPEVTCVVVDVSQEDPEVQFNWYVDGVEVHNAKTKPREEQFNSTYRVVSVLTVLHQDWLNGKEYKCKVSNKGLPSSIEKTISKAKGQPREPQVYTLPPSQEEMTKNQVSLTCLVKGFYPSDIAVEWESNGQPENNYKTTPPVLDSDGSFFLYSRLTVDKSRWQEGNVFSCSVMHEALHNHYTQKSLSLSLGK

SEQ ID NO: 98 - protein, 960 aa, synthetic construct
QVQLVQSGAEVKKPGSSVKVSCKASGGTFSSYAISWVRQAPGQGLEWMGGIIPIFGTANYAQKFQGRVTITADESTSTAYMELSSLRSEDTAVYYCARGLWEVRALPSVYWGQGTLVTVSSSSSSGSSSSGSSSSGSYELTQPPSVSVAPGQTARITCGANDIGSKSVHWYQQKAGQAPVLVVSEDIIRPSGIPERISGSNSGNTATLTISRVEAGDEADYYCQVWDRDSDQYVFGTGTKVTVLGGGGSGGGGSGGGGSEVQLLESGGGLVQPGGSLRLSCAASGFTFSSFSMSWVRQAPGKGLEWVSSISGSSGTTYYADSVKGRFTISRDNSKNTLYLQMNSLRAEDTAVYYCAKPFPYFDYWGQGTLVTVSSGGGGSGGGGSGGGGSEIVLTQSPGTLSLSPGERATLSCRASQSVSSSFLAWYQQKPGQAPRLLIYYASSRATGIPDRFSGSGSGTDFTLTISRLEPEDFAVYYCQQTGRIPPTFGQGTKVEIKSSSSGSSSSGSSSSGQVQLVQSGVEVKKPGASVKVSCKASGYTFTNYYMYWVRQAPGQGLEWMGGINPSNGGTNFNEKFKNRVTLTTDSSTTTAYMELKSLQFDDTAVYYCARRDYRFDMGFDYWGQGTTVTVSSASTKGPSVFPLAPCSRSTSESTAALGCLVKDYFPEPVTVSWNSGALTSGVHTFPAVLQSSGLYSLSSVVTVPSSSLGTKTYTCNVDHKPSNTKVDKRVESKYGPPCPPCPAPEFLGGPSVFLFPPKPKDTLMISRTPEVTCVVVDVSQEDPEVQFNWYVDGVEVHNAKTKPREEQFNSTYRVVSVLTVLHQDWLNGKEYKCKVSNKGLPSSIEKTISKAKGQPREPQVYTLPPSQEEMTKNQVSLTCLVKGFYPSDIAVEWESNGQPENNYKTTPPVLDSDGSFFLYSRLTVDKSRWQEGNVFSCSVMHEALHNHYTQKSLSLSLGK

SEQ ID NO: 99 - protein, 1003 aa, synthetic construct
QVQLVQSGVEVKKPGASVKVSCKASGYTFTNYYMYWVRQAPGQGLEWMGGINPSNGGTNFNEKFKNRVTLTTDSSTTTAYMELKSLQFDDTAVYYCARRDYRFDMGFDYWGQGTTVTVSSGGGGSGGGGSGGGGSEIVLTQSPATLSLSPGERATLSCRASKGVSTSGYSYLHWYQQKPGQAPRLLIYLASYLESGVPARFSGSGSGTDFTLTISSLEPEDFAVYYCQHSRDLPLTFGGGTKVEIKSSSSGSSSSGSSSSGESKYGPPCPPCPAPEFLGGPSVFLFPPKPKDTLMISRTPEVTCVVVDVSQEDPEVQFNWYVDGVEVHNAKTKPREEQFNSTYRVVSVLTVLHQDWLNGKEYKCKVSNKGLPSSIEKTISKAKGQPREPQVYTLPPSQEEMTKNQVSLTCLVKGFYPSDIAVEWESNGQPENNYKTTPPVLDSDGSFFLYSRLTVDKSRWQEGNVFSCSVMHEALHNHYTQKSLSLSLGKGGGGSGGGGSGGGGSEVQLLESGGGLVQPGGSLRLSCAASGFTFSSFSMSWVRQAPGKGLEWVSSISGSSGTTYYADSVKGRFTISRDNSKNTLYLQMNSLRAEDTAVYYCAKPFPYFDYWGQGTLVTVSSGGGGSGGGGSGGGGSEIVLTQSPGTLSLSPGERATLSCRASQSVSSSFLAWYQQKPGQAPRLLIYYASSRATGIPDRFSGSGSGTDFTLTISRLEPEDFAVYYCQQTGRIPPTFGQGTKVEIKGGGGSGGGGSGGGGSQVQLVQSGAEVKKPGSSVKVSCKASGGTFSSYAISWVRQAPGQGLEWMGGIIPIFGTANYAQKFQGRVTITADESTSTAYMELSSLRSEDTAVYYCARGLWEVRALPSVYWGQGTLVTVSSSSSSGSSSSGSSSSGSYELTQPPSVSVAPGQTARITCGANDIGSKSVHWYQQKAGQAPVLVVSEDIIRPSGIPERISGSNSGNTATLTISRVEAGDEADYYCQVWDRDSDQYVFGTGTKVTVL

SEQ ID NO: 100 - protein, 1003 aa, synthetic construct
QVQLVQSGVEVKKPGASVKVSCKASGYTFTNYYMYWVRQAPGQGLEWMGGINPSNGGTNFNEKFKNRVTLTTDSSTTTAYMELKSLQFDDTAVYYCARRDYRFDMGFDYWGQGTTVTVSSGGGGSGGGGSGGGGSEIVLTQSPATLSLSPGERATLSCRASKGVSTSGYSYLHWYQQKPGQAPRLLIYLASYLESGVPARFSGSGSGTDFTLTISSLEPEDFAVYYCQHSRDLPLTFGGGTKVEIKSSSSGSSSSGSSSSGESKYGPPCPPCPAPEFLGGPSVFLFPPKPKDTLMISRTPEVTCVVVDVSQEDPEVQFNWYVDGVEVHNAKTKPREEQFNSTYRVVSVLTVLHQDWLNGKEYKCKVSNKGLPSSIEKTISKAKGQPREPQVYTLPPSQEEMTKNQVSLTCLVKGFYPSDIAVEWESNGQPENNYKTTPPVLDSDGSFFLYSRLTVDKSRWQEGNVFSCSVMHEALHNHYTQKSLSLSLGKGGGGSGGGGSGGGGSQVQLVQSGAEVKKPGSSVKVSCKASGGTFSSYAISWVRQAPGQGLEWMGGIIPIFGTANYAQKFQGRVTITADESTSTAYMELSSLRSEDTAVYYCARGLWEVRALPSVYWGQGTLVTVSSSSSSGSSSSGSSSSGSYELTQPPSVSVAPGQTARITCGANDIGSKSVHWYQQKAGQAPVLVVSEDIIRPSGIPERISGSNSGNTATLTISRVEAGDEADYYCQVWDRDSDQYVFGTGTKVTVLGGGGSGGGGSGGGGSEVQLLESGGGLVQPGGSLRLSCAASGFTFSSFSMSWVRQAPGKGLEWVSSISGSSGTTYYADSVKGRFTISRDNSKNTLYLQMNSLRAEDTAVYYCAKPFPYFDYWGQGTLVTVSSGGGGSGGGGSGGGGSEIVLTQSPGTLSLSPGERATLSCRASQSVSSSFLAWYQQKPGQAPRLLIYYASSRATGIPDRFSGSGSGTDFTLTISRLEPEDFAVYYCQQTGRIPPTFGQGTKVEIK

SEQ ID NO: 101 - protein, 1003 aa, synthetic construct
EVQLLESGGGLVQPGGSLRLSCAASGFTFSSFSMSWVRQAPGKGLEWVSSISGSSGTTYYADSVKGRFTISRDNSKNTLYLQMNSLRAEDTAVYYCAKPFPYFDYWGQGTLVTVSSGGGGSGGGGSGGGGSEIVLTQSPGTLSLSPGERATLSCRASQSVSSSFLAWYQQKPGQAPRLLIYYASSRATGIPDRFSGSGSGTDFTLTISRLEPEDFAVYYCQQTGRIPPTFGQGTKVEIKGGGGSGGGGSGGGGSQVQLVQSGAEVKKPGSSVKVSCKASGGTFSSYAISWVRQAPGQGLEWMGGIIPIFGTANYAQKFQGRVTITADESTSTAYMELSSLRSEDTAVYYCARGLWEVRALPSVYWGQGTLVTVSSSSSSGSSSSGSSSSGSYELTQPPSVSVAPGQTARITCGANDIGSKSVHWYQQKAGQAPVLVVSEDIIRPSGIPERISGSNSGNTATLTISRVEAGDEADYYCQVWDRDSDQYVFGTGTKVTVLGGGGSGGGGSGGGGSESKYGPPCPPCPAPEFLGGPSVFLFPPKPKDTLMISRTPEVTCVVVDVSQEDPEVQFNWYVDGVEVHNAKTKPREEQFNSTYRVVSVLTVLHQDWLNGKEYKCKVSNKGLPSSIEKTISKAKGQPREPQVYTLPPSQEEMTKNQVSLTCLVKGFYPSDIAVEWESNGQPENNYKTTPPVLDSDGSFFLYSRLTVDKSRWQEGNVFSCSVMHEALHNHYTQKSLSLSLGKSSSSGSSSSGSSSSGQVQLVQSGVEVKKPGASVKVSCKASGYTFTNYYMYWVRQAPGQGLEWMGGINPSNGGTNFNEKFKNRVTLTTDSSTTTAYMELKSLQFDDTAVYYCARRDYRFDMGFDYWGQGTTVTVSSGGGGSGGGGSGGGGSEIVLTQSPATLSLSPGERATLSCRASKGVSTSGYSYLHWYQQKPGQAPRLLIYLASYLESGVPARFSGSGSGTDFTLTISSLEPEDFAVYYCQHSRDLPLTFGGGTKVEIK

SEQ ID NO: 102 - protein, 759 aa, synthetic construct
QVQLVQSGVEVKKPGASVKVSCKASGYTFTNYYMYWVRQAPGQGLEWMGGINPSNGGTNFNEKFKNRVTLTTDSSTTTAYMELKSLQFDDTAVYYCARRDYRFDMGFDYWGQGTTVTVSSGGGGSGGGGSGGGGSEIVLTQSPATLSLSPGERATLSCRASKGVSTSGYSYLHWYQQKPGQAPRLLIYLASYLESGVPARFSGSGSGTDFTLTISSLEPEDFAVYYCQHSRDLPLTFGGGTKVEIKSSSSGSSSSGSSSSGEVQLLESGGGLVQPGGSLRLSCAASGFTFSSFSMSWVRQAPGKGLEWVSSISGSSGTTYYADSVKGRFTISRDNSKNTLYLQMNSLRAEDTAVYYCAKPFPYFDYWGQGTLVTVSSGGGGSGGGGSGGGGSEIVLTQSPGTLSLSPGERATLSCRASQSVSSSFLAWYQQKPGQAPRLLIYYASSRATGIPDRFSGSGSGTDFTLTISRLEPEDFAVYYCQQTGRIPPTFGQGTKVEIKGGGGSGGGGSGGGGSQVQLVQSGAEVKKPGSSVKVSCKASGGTFSSYAISWVRQAPGQGLEWMGGIIPIFGTANYAQKFQGRVTITADESTSTAYMELSSLRSEDTAVYYCARGLWEVRALPSVYWGQGTLVTVSSSSSSGSSSSGSSSSGSYELTQPPSVSVAPGQTARITCGANDIGSKSVHWYQQKAGQAPVLVVSEDIIRPSGIPERISGSNSGNTATLTISRVEAGDEADYYCQVWDRDSDQYVFGTGTKVTVL

SEQ ID NO: 103 - protein, 759 aa, synthetic construct
QVQLVQSGVEVKKPGASVKVSCKASGYTFTNYYMYWVRQAPGQGLEWMGGINPSNGGTNFNEKFKNRVTLTTDSSTTTAYMELKSLQFDDTAVYYCARRDYRFDMGFDYWGQGTTVTVSSGGGGSGGGGSGGGGSEIVLTQSPATLSLSPGERATLSCRASKGVSTSGYSYLHWYQQKPGQAPRLLIYLASYLESGVPARFSGSGSGTDFTLTISSLEPEDFAVYYCQHSRDLPLTFGGGTKVEIKSSSSGSSSSGSSSSGQVQLVQSGAEVKKPGSSVKVSCKASGGTFSSYAISWVRQAPGQGLEWMGGIIPIFGTANYAQKFQGRVTITADESTSTAYMELSSLRSEDTAVYYCARGLWEVRALPSVYWGQGTLVTVSSSSSSGSSSSGSSSSGSYELTQPPSVSVAPGQTARITCGANDIGSKSVHWYQQKAGQAPVLVVSEDIIRPSGIPERISGSNSGNTATLTISRVEAGDEADYYCQVWDRDSDQYVFGTGTKVTVLGGGGSGGGGSGGGGSEVQLLESGGGLVQPGGSLRLSCAASGFTFSSFSMSWVRQAPGKGLEWVSSISGSSGTTYYADSVKGRFTISRDNSKNTLYLQMNSLRAEDTAVYYCAKPFPYFDYWGQGTLVTVSSGGGGSGGGGSGGGGSEIVLTQSPGTLSLSPGERATLSCRASQSVSSSFLAWYQQKPGQAPRLLIYYASSRATGIPDRFSGSGSGTDFTLTISRLEPEDFAVYYCQQTGRIPPTFGQGTKVEIK

SEQ ID NO: 104 - protein, 759 aa, synthetic construct
QVQLVQSGAEVKKPGSSVKVSCKASGGTFSSYAISWVRQAPGQGLEWMGGIIPIFGTANYAQKFQGRVTITADESTSTAYMELSSLRSEDTAVYYCARGLWEVRALPSVYWGQGTLVTVSSSSSSGSSSSGSSSSGSYELTQPPSVSVAPGQTARITCGANDIGSKSVHWYQQKAGQAPVLVVSEDIIRPSGIPERISGSNSGNTATLTISRVEAGDEADYYCQVWDRDSDQYVFGTGTKVTVLGGGGSGGGGSGGGGSEVQLLESGGGLVQPGGSLRLSCAASGFTFSSFSMSWVRQAPGKGLEWVSSISGSSGTTYYADSVKGRFTISRDNSKNTLYLQMNSLRAEDTAVYYCAKPFPYFDYWGQGTLVTVSSGGGGSGGGGSGGGGSEIVLTQSPGTLSLSPGERATLSCRASQSVSSSFLAWYQQKPGQAPRLLIYYASSRATGIPDRFSGSGSGTDFTLTISRLEPEDFAVYYCQQTGRIPPTFGQGTKVEIKSSSSGSSSSGSSSSGQVQLVQSGVEVKKPGASVKVSCKASGYTFTNYYMYWVRQAPGQGLEWMGGINPSNGGTNFNEKFKNRVTLTTDSSTTTAYMELKSLQFDDTAVYYCARRDYRFDMGFDYWGQGTTVTVSSGGGGSGGGGSGGGGSEIVLTQSPATLSLSPGERATLSCRASKGVSTSGYSYLHWYQQKPGQAPRLLIYLASYLESGVPARFSGSGSGTDFTLTISSLEPEDFAVYYCQHSRDLPLTFGGGTKVEIK

SEQ ID NO: 105 - protein, 381 aa, synthetic construct
IPPHVQKSVNNDMIVTDNNGAVKFPQLCKFCDVRFSTCDNQKSCMSNCSITSICEKPQEVCVAVWRKNDENITLETVCHDPKLPYHDFILEDAASPKCIMKEKKKPGETFFMCSCSSDECNDNIIFSEEYNTSNPDGGGGGSGGGGSGGGGSESKYGPPCPPCPAPEFLGGPSVFLFPPKPKDTLMISRTPEVTCVVVDVSQEDPEVQFNWYVDGVEVHNAKTKPREEQFNSTYRVVSVLTVLHQDWLNGKEYKCKVSNKGLPSSIEKTISKAKGQPREPQVYTLPPSQEEMTKNQVSLTCLVKGFYPSDIAVEWESNGQPENNYKTTPPVLDSDGSFFLYSRLTVDKSRWQEGNVFSCSVMHEALHNHYTQKSLSLSLGK

SEQ ID NO: 106 - protein, 380 aa, synthetic construct
ESKYGPPCPPCPAPEFLGGPSVFLFPPKPKDTLMISRTPEVTCVVVDVSQEDPEVQFNWYVDGVEVHNAKTKPREEQFNSTYRVVSVLTVLHQDWLNGKEYKCKVSNKGLPSSIEKTISKAKGQPREPQVYTLPPSQEEMTKNQVSLTCLVKGFYPSDIAVEWESNGQPENNYKTTPPVLDSDGSFFLYSRLTVDKSRWQEGNVFSCSVMHEALHNHYTQKSLSLSLGKGGGGSGGGGSGGGGSIPPHVQKSVNNDMIVTDNNGAVKFPQLCKFCDVRFSTCDNQKSCMSNCSITSICEKPQEVCVAVWRKNDENITLETVCHDPKLPYHDFILEDAASPKCIMKEKKKPGETFFMCSCSSDECNDNIIFSEEYNTSNPD

SEQ ID NO: 107 - protein, 265 aa, synthetic construct
ESKYGPPCPPCPAPEFLGGPSVFLFPPKPKDTLMISRTPEVTCVVVDVSQEDPEVQFNWYVDGVEVHNAKTKPREEQFNSTYRVVSVLTVLHQDWLNGKEYKCKVSNKGLPSSIEKTISKAKGQPREPQVYTLPPSQEEMTKNQVSLTCLVKGFYPSDIAVEWESNGQPENNYKTTPPVLDSDGSFFLYSRLTVDKSRWQEGNVFSCSVMHEALHNHYTQKSLSLSLGKGGGGSGGGGSSSSPIQGSWTWENGKWTWKGIIRLEQ

SEQ ID NO: 108 - protein, 442 aa, synthetic construct
EVQLLESGGGLVQPGGSLRLSCAASGFTFSSFSMSWVRQAPGKGLEWVSSISGSSGTTYYADSVKGRFTISRDNSKNTLYLQMNSLRAEDTAVYYCAKPFPYFDYWGQGTLVTVSSASTKGPSVFPLAPCSRSTSESTAALGCLVKDYFPEPVTVSWNSGALTSGVHTFPAVLQSSGLYSLSSVVTVPSSSLGTKTYTCNVDHKPSNTKVDKRVESKYGPPCPPCPAPEFLGGPSVFLFPPKPKDTLMISRTPEVTCVVVDVSQEDPEVQFNWYVDGVEVHNAKTKPREEQFNSTYRVVSVLTVLHQDWLNGKEYKCKVSNKGLPSSIEKTISKAKGQPREQVYTLPPSQEEMTKNQVSLTCLVKGFYPSDIAVEWESNGQPENNYKTTPPVLDSDGSFFLYSRLTVDKSRWQEGNVFSCSVMHEALHNHYTQKSLSLSLGK

SEQ ID NO: 109 - protein, 447 aa, synthetic construct
QVQLVQSGVEVKKPGASVKVSCKASGYTFTNYYMYWVRQAPGQGLEWMGGINPSNGGTNFNEKFKNRVTLTTDSSTTTAYMELKSLQFDDTAVYYCARRDYRFDMGFDYWGQGTTVTVSSASTKGPSVFPLAPCSRSTSESTAALGCLVKDYFPEPVTVSWNSGALTSGVHTFPAVLQSSGLYSLSSVVTVPSSSLGTKTYTCNVDHKPSNTKVDKRVESKYGPPCPPCPAPEFLGGPSVFLFPPKPKDTLMISRTPEVTCVVVDVSQEDPEVQFNWYVDGVEVHNAKTKPREEQFNSTYRVVSVLTVLHQDWLNGKEYKCKVSNKGLPSSIEKTISKAKGQPREPQVYTLPPSQEEMTKNQVSLTCLVKGFYPSDIAVEWESNGQPENNYKTTPPVLDSDGSFFLYSRLTVDKSRWQEGNVFSCSVMHEALHNHYTQKSLSLSLGK

SEQ ID NO: 110 - skipped

SEQ ID NO: 111 - protein, 5 aa, synthetic construct
GGGGS

SEQ ID NO: 112 - protein, 5 aa, synthetic construct
SSSSG

SEQ ID NO: 113 - protein, 180 aa, synthetic construct
SSCTFDNLSPGLEYNVSVYTVKDDKESVPISDTIIPEVPQLTDLSFVDITDSSIGLRWTPLNSSTIIGYRITVVAAGEGIPIFEDFVDSSVGYYTVTGLEPGIDYDISVITLINGGESAPTTLTQQTAVPPPTDLRFTNIGPDTMRVTWAPPPSIDLTNFLVRYSPVKNEEDVAELSISP

SEQ ID NO: 114 - protein, 180 aa, synthetic construct; identical to SEQ ID NO: 113

SEQ ID NO: 115 - protein, 180 aa, synthetic construct
SSCTFENLNPGLEYNVSVYTVKDDKESAPISDTVIPEVPQLTDLSFVDITDSSIGLRWTPLNSSTIIGYRITVVAAGEGIPIFEDFVDSSVGYYTVTGLEPGIDYDISVITLINGGESAPTTLTQQTAVPPPTDLRFTNIGPDTMRVTWAPPPSIELTNLLVRYSPVKNEEDVAELSISP

SEQ ID NO: 116 - protein, 180 aa, synthetic construct
SSCTFENLNPGLEYNVSVYTVKDDKESAPISDTVVPEVPQLTDLSFVDITDSSIGLRWTPLNSSTIIGYRITVVAAGEGIPIFEDFVDSSVGYYTVTGLEPGIDYDISVITLINGGESAPTTLTQQTAVPPPTDLRFTNIGPDTMRVTWAPPPSIELTNLLVRYSPVKNEEDVAELSISP

SEQ ID NO: 117 - protein, 19 aa, synthetic construct
MGWSCIILFLVATATGAYA